European Patent Specification EP 3 185 909 B1, published April 3, 2024. Title: METHODS AND COMPOSITIONS FOR TREATING LEBER CONGENITAL AMAUROSIS. Applicant: The United States of America, as represented by the Secretary, Department of Health and Human Services Wu, Zhijian Swaroop, Anand Mookherjee, Suddhasil Hiriyanna, Suja. Application not yet assigned. The sequence listing filed with the application follows.

SEQUENCE LISTING (45 sequences)

SEQ ID NO: 1 - DNA, 7440 bp, Mus musculus
atgccacctaatataaagtggaaagaattaatcaaagttgatccagatgacctgccacggcaagaagagttagcagataaattattgatatctttatccaaggtggaagtaaatgaactaaaaaatgaagaccaagaaaacatgatacatctattcagaattacccagtctctaatgaagatgaaagcccaggaagtagagctcgctttggaagaagttgaaaaggctggagaagaacaagcaaaatttgaaaatcaattaaagacaaaagtaatgaaactggaaaatgaactggagatggctcagcagtctgcagggggacgtgacactcggtttttacgtgacgaaattcgccaacttgagaagcagctggaacaaaaagatagagaattagaggatatggaaaaagaattggataaagaaaagaaggttaatgaacaattggctcttcgaaatgaggaggcagaaaatgaaaacagcaaattaagaagagagaacaaacgtctaaagaaaaagaatgagcagcttcggcaggacattattgactaccagaaacaaatagattcacagaaagaatcacttctgtcaaggagaggagaagacagtgactaccgatcacagttgtctaaaaagaactatgaacttgttcaatatctggacgaaatacagaccttaacagaagctaatgagaagattgaagttcagaaccaagaaatgaggaaaaacctggaagagtctgtgcaggagatggagaagatgactgatgagtacaacaggatgaaagcgcttgtgcatcagtcggatgctgtcatggaccagatcaagaaggagaatgagcactatcgcctgcaagttcgagagctcacggatcttctgaaggcgaaggatgaagaggacgatccagtcatgatggctgttaacgcaaaagtggaagagtggaagttaattttgtcttctaaagatgatgaaatcattgaatatcagcaaatgctacagagtctgagagggaaacttaaaaatgcccaacttgatgcagacaaaagtaacatcatggctctgaaacagggtatccaggagcgagacagtcaaattaagatgcttactgagcaagtagaacagtatacgaaagaaatggaaaaaaatacgtttattattgaagatttgaaaaatgaactccaaaaagacaaaggtacttcaaacttttatcagcagactcattatatgaaaattcactcaaaagtacaaattttagaagagaaaacaaaagaggccgagagaatagctgagctggctgaggctgatgccagggagaaggacaaagaattggttgaggctctgaagagattaaaagattatgaatctggagtatatggcttagaagatgctgttatcgaaataaagaattgtaaagcccaaattaaaataagagatggagagatggaagtgttgaccaaggagatcaataagcttgagatgaagatcaatgacatccttgatgaaaacgaagcccttagagagcgggctggccttgaacccaagacaatgattgatttgactgaatttagaaacagcaaacggttaaagcagcaacagtacagagctgagaaccaggttcttttgaaagagatcgaaagtctagaggaggagcgtcttgacttgaaaagaaagattcgtcaaatggctcaagaaagaggcaaaaggaacgcagcctcaggattaaccattgacgacttgaacttatctgaaaccttttctcatgaaaataaaatagaaggaagaaaactaaattttatgagcctcaataatatgaatgaaacacaatcaaagaatgagtttctttcaagagaattggctgaaaaggaaaaagatttagaaagaagtaggacagtaattgctaaattccagagtaaactaaaagaattagtcgaagaaaataagcaacttgaagaaggtatgaaagaaattttgcaagctattaaggacatgccgaaggattctgatgtgaaaggaggtgaaacatctttaatcatcccgagtcttgaaagactggttaacgctatggaatcaaagaatgcagaaggaatcttcgatgccagcttgcatctaaaagcccaagttgaccaacttacaggaaggaatgaagaattaaggcaagaactcaggcaatctcggaaagaggctgtaaattattcacagcagttggtaaaagcaaacttaaagattgaccaccttgagaaggaaactgaccttctacgtcagtctgcaggctccaatgtagtatacaaaggcatagacttacccgatgggatagcaccatccagtgcctatatcatcaattctcagaatgaatacttaatacatcttttgcaggaactagacaataaagaaaagaaattaaaacatttagaagattcccttgaagattataacagaaagtttgcagtgattcgtcatcaacaaagtttattatataaagaatacctaagtgaaaaggatatttggaaaacagactctgagatgataagagaggagaagagaaaactggaagatcaagctgagcaggatgctgtgaaagtaaaagagtacaacaatttgctcagtgctcttcagatggattcgaacgagatgaagaaaatgctctcagaaaacagtaggaaaatcaccgttctgcaagtgaacgagaagtccctcatccggcagtacaccaccttagtggagatggagcggcacctgagaaaggaaaacgggaaacacaggaatgacgtcatagccatggaggccgaagtcactgaaaaacttggaagtttgcaaagattcaaggaaatggccatcttcaagattgcagctcttcagaaggttatagataatagtgtttctttgtctgaattagaactagccaataaacagtacaatgagctgactactaagtacagggacatcttgcagaaagataatatgcttgttcaaagaacaagtaacttagaacacctggagtgtgagaatgcatcgctaaaagaacagatggaggctatcagtaaagagctggagattacaaaggaaaaactccataccattgaacaggcctgggaacaagaaacgaagttaggaaatgactcaaacatggataaggctaagaaatcaatgacaaacagtgacattgtttctatttcaaagaaaatcactgtgttggagatgaaggaattaaatgaaaggcagagggctgaacactgtcagaaaatgtatgagcacttaaggacttcattaaagcaaatggaagaacgtaattttgaattggaaaccaagttcactgagcttactaaaatcaacctggatgcacaaaaggtggagcagatgttgagagacgaattagctgatagtgtgaccaaggcagtaagtgatgctgaccgacagcggattctagaactagagaagagtgaagtggagctcaaagttgaagtgtccaagctgagagagatttcagatattgccaaaagacaagttgattttttgaattcgcaacaacagtccagggaaaaggaagtggaatccctcagaacgcagctgctggacttccaggcacaatctgacgaaaaggctctaattgccaaattgcaccaacatgttgtctctcttcaaattagtgaggccactgccctcggtaagttagagtcagttacgtccaaactccagaagatggaagcctacaatttgcgcttagaacagaaactggatgaaaaagagcaggcgctctactatgctcgtttggaaggtagaaacagagcaaaacacctgcgccaaaccattcagtcgcttcgaagacagttcagtggagctctacccttagcacagcaggaaaagttctccaaaacgatgattcagttgcaaaatgacaaacttaagataatgcaagaaatgaagaattcgcaacaggaacacagaaatatggaaaacaaaacactggagttggaattaaaattaaaaggcttagaagaattgatcagtactttaaaggatgccaggggagcccagaaggtaatcaattggcatgtgaaaatagaagaacttcgcctccaagaacttaagctaaatagagaactagtcaagggtaaagaagaaatcaaatatttgaataatatcatctctgaatatgagcatacaatcaacagtctagaggaagaaattgttcagcaaagcaagttccatgaagaaagacagatggcttgggatcaaagagaagttgagctggaacgccagttagacatttttgatcatcagcaaaatgaaatactcagtgcagcacaaaagtttgaagactctacaggatcaatgccagaccccagcttgcctcttccaaaccaacttgaaattgctctaagaaaaattaaggagaatattcaagtaattcttaaaacacaagcaacttgcaagtcactagaagagaaactaaaagaaaaagaatctgctttacggttggcagagcaaaatattctgtcaagagacaaagtaatcaatgaactgaggcttcgattgcctgccacggctgatcgagaaaaacttatagctgagctagaaagaaaagagctggagccgaaatctcatcacacaatgaaaattgcccaccaaactattgccaacatgcaggcaaggttaaatcacaaggaagaagtattgaagaaataccagcaccttctggagaaggccagagaggagcaaagagaaattgttaagaagcatgaggaagaccttcatgttcttcatcacaaattagaacaacaggccgataattcactcaataaattcagacagacagctcaggatttacttaagcagtctcctgctccagttcccaccaacaaacatttcattcgtctggccgagatggagcagacagtagcagaacaagatgactctctgtcctcacttttgaccaaactaaagaaagtatcaaaagatttggaaaaacaaaaagaaatcactgagttaaaagtcagagagtttgaaaataccaaactacggctccaagaaactcatgccagtgaggtaaagaaagtgaaagcagaggtagaggacttaaggcatgctctagcccaagcacacaaggactcccagagtttaaagtctgaactccaggctcagaaagaagcaaactccagagctccaacaaccacaatgaggaatcttgtagacaggctaaagagccaactagccttgaaagagaagcaacaaaaggcacttagtcgagccctgttggaacttcggtcggaaatgacagcagcagctgaggaacgtataatcgctgtaacttctcaaaaagaggcaaatctcaatgttcaacaagttgttgagcgccatactagagagctaaagtcacaaattgaagatttaaatgaaaatcttttaaaattgaaagaagctcttaaaacaagtaagaacaaagaaaattcactagctgatgatttaaatgaattaaataatgaactgcaaaaaaagcaaaaagcttataataaaatccttagagagaaagatggaattgatcaagaaaatgatgaactgagaagacagattaaaagactgtccagtggactgcagagcaaaactttgatagataacaagcaaagtttaatcgatgaacttcaaaagaaagttaaaaaacttgaaagccaactggaaagaaaggtggatgacgtagacataaagccggtgaaggaaaagagtagtaaagaagaattaattaggtgggaagaaggtaagaaatggcaaaccaaagtagagggactacgaaacagactaaaggagaaggaaggagaagcccacggcctggcaaagcagctgaataccttaaaggaactttttgccaaagctgataaagagaaacttactttgcagaagaaactgaaaacaacaggaatgactgttgaccaggttttaggagtgcgagctttggaatctgaaaaagagttggaagagctaaaaaagaaaaatctggacctagaaaatgacatattatacatgaggacccagcaggctcttccacgagattctgttgtggaagacttacatttacaaaataaataccttcaagaaaaacttcatactttagaaaaaaaactttcaaaggagaaatattctcagtctttgacttcagaaatagagtcagatgatcactgtcaaaaagaacaagaacttcagaaggaaaatttgaagttgtcatctgaaaacatcgagctgaaatttcaacttgaacaagcaaataaagatttgccaagactaaagaatcaagtgaaagatttgaaggaaatgtgtgaatttcttaagaaaggaaaactggaacttgagcggaagcttggtcaggtcagaggggctggtagaagtgggaagacaatcccagaactagaaaaaaccattgggttaatgaagaaagtagttgaaaaagtccaaagagaaaatgaacaattgaaaaaggcatcaggaatactgactagtgaaaaaatggctactattgaggaagaaaatagaaacttaaaggctgaactagaaaagcttaaagctcactttggacgtcagttgagtatgcagtttgaatctaagaacaaaggtactgagaaaattgttgccgaaaatgaacggcttcggaaagaacttaagaaagaaatagaagcctctgagaaactgcggatagctaagaacaacttagagctggtgaacgacaagatggcagctcaactcgaagaaactgggaagagactacagtttgcagaaagtagagccccacagctggaaggtgctgacagcaagagctggaagtcaattgtggtctcaagagtgtatgagaccaagatgaaagagcttgaaagtgacattgccaaaaagaatcaaagtatcactgaccttaaacagcttgtaagagaagcaacagagagagaacagaaagctaagaaatacactgaagaccttgaacaacagattgagatcctcaaaaatgttcctgaaggtgccgagacagagcaagagcttatacgggaactccagcttcttagattagccaataatcagatggataaagaaagggcagaattaatccatcagatagaaattaacaaggaccaaaccagagctgacagtagcatacctgattctgatcaactaaaggaaaagataaatgacctggagacacaactcagaaagttggagctagaaaagcaacattcgaaggaggaagttaaaaagctgaaaaaagaactggaaaattttgatccttcattttttgaagaaattgaagacctgaagtataattataaggaagaagtgaaaaagaatatcctattagaagagaagctaaaaaaactgtcggaacagtttggatttgaactgcctagtcctcttgctgcttctgaacactcggaagatggagaaagtcctcatagtttccctatttattag

SEQ ID NO: 2 - protein, 2479 aa, Mus musculus
MPPNIKWKELIKVDPDDLPRQEELADKLLISLSKVEVNELKNEDQENMIHLFRITQSLMKMKAQEVELALEEVEKAGEEQAKFENQLKTKVMKLENELEMAQQSAGGRDTRFLRDEIRQLEKQLEQKDRELEDMEKELDKEKKVNEQLALRNEEAENENSKLRRENKRLKKKNEQLRQDIIDYQKQIDSQKESLLSRRGEDSDYRSQLSKKNYELVQYLDEIQTLTEANEKIEVQNQEMRKNLEESVQEMEKMTDEYNRMKALVHQSDAVMDQIKKENEHYRLQVRELTDLLKAKDEEDDPVMMAVNAKVEEWKLILSSKDDEIIEYQQMLQSLRGKLKNAQLDADKSNIMALKQGIQERDSQIKMLTEQVEQYTKEMEKNTFIIEDLKNELQKDKGTSNFYQQTHYMKIHSKVQILEEKTKEAERIAELAEADAREKDKELVEALKRLKDYESGVYGLEDAVIEIKNCKAQIKIRDGEMEVLTKEINKLEMKINDILDENEALRERAGLEPKTMIDLTEFRNSKRLKQQQYRAENQVLLKEIESLEEERLDLKRKIRQMAQERGKRNAASGLTIDDLNLSETFSHENKIEGRKLNFMSLNNMNETQSKNEFLSRELAEKEKDLERSRTVIAKFQSKLKELVEENKQLEEGMKEILQAIKDMPKDSDVKGGETSLIIPSLERLVNAMESKNAEGIFDASLHLKAQVDQLTGRNEELRQELRQSRKEAVNYSQQLVKANLKIDHLEKETDLLRQSAGSNVVYKGIDLPDGIAPSSAYIINSQNEYLIHLLQELDNKEKKLKHLEDSLEDYNRKFAVIRHQQSLLYKEYLSEKDIWKTDSEMIREEKRKLEDQAEQDAVKVKEYNNLLSALQMDSNEMKKMLSENSRKITVLQVNEKSLIRQYTTLVEMERHLRKENGKHRNDVIAMEAEVTEKLGSLQRFKEMAIFKIAALQKVIDNSVSLSELELANKQYNELTTKYRDILQKDNMLVQRTSNLEHLECENASLKEQMEAISKELEITKEKLHTIEQAWEQETKLGNDSNMDKAKKSMTNSDIVSISKKITVLEMKELNERQRAEHCQKMYEHLRTSLKQMEERNFELETKFTELTKINLDAQKVEQMLRDELADSVTKAVSDADRQRILELEKSEVELKVEVSKLREISDIAKRQVDFLNSQQQSREKEVESLRTQLLDFQAQSDEKALIAKLHQHVVSLQISEATALGKLESVTSKLQKMEAYNLRLEQKLDEKEQALYYARLEGRNRAKHLRQTIQSLRRQFSGALPLAQQEKFSKTMIQLQNDKLKIMQEMKNSQQEHRNMENKTLELELKLKGLEELISTLKDARGAQKVINWHVKIEELRLQELKLNRELVKGKEEIKYLNNIISEYEHTINSLEEEIVQQSKFHEERQMAWDQREVELERQLDIFDHQQNEILSAAQKFEDSTGSMPDPSLPLPNQLEIALRKIKENIQVILKTQATCKSLEEKLKEKESALRLAEQNILSRDKVINELRLRLPATADREKLIAELERKELEPKSHHTMKIAHQTIANMQARLNHKEEVLKKYQHLLEKAREEQREIVKKHEEDLHVLHHKLEQQADNSLNKFRQTAQDLLKQSPAPVPTNKHFIRLAEMEQTVAEQDDSLSSLLTKLKKVSKDLEKQKEITELKVREFENTKLRLQETHASEVKKVKAEVEDLRHALAQAHKDSQSLKSELQAQKEANSRAPTTTMRNLVDRLKSQLALKEKQQKALSRALLELRSEMTAAAEERIIAVTSQKEANLNVQQVVERHTRELKSQIEDLNENLLKLKEALKTSKNKENSLADDLNELNNELQKKQKAYNKILREKDGIDQENDELRRQIKRLSSGLQSKTLIDNKQSLIDELQKKVKKLESQLERKVDDVDIKPVKEKSSKEELIRWEEGKKWQTKVEGLRNRLKEKEGEAHGLAKQLNTLKELFAKADKEKLTLQKKLKTTGMTVDQVLGVRALESEKELEELKKKNLDLENDILYMRTQQALPRDSVVEDLHLQNKYLQEKLHTLEKKLSKEKYSQSLTSEIESDDHCQKEQELQKENLKLSSENIELKFQLEQANKDLPRLKNQVKDLKEMCEFLKKGKLELERKLGQVRGAGRSGKTIPELEKTIGLMKKVVEKVQRENEQLKKASGILTSEKMATIEEENRNLKAELEKLKAHFGRQLSMQFESKNKGTEKIVAENERLRKELKKEIEASEKLRIAKNNLELVNDKMAAQLEETGKRLQFAESRAPQLEGADSKSWKSIVVSRVYETKMKELESDIAKKNQSITDLKQLVREATEREQKAKKYTEDLEQQIEILKNVPEGAETEQELIRELQLLRLANNQMDKERAELIHQIEINKDQTRADSSIPDSDQLKEKINDLETQLRKLELEKQHSKEEVKKLKKELENFDPSFFEEIEDLKYNYKEEVKKNILLEEKLKKLSEQFGFELPSPLAASEHSEDGESPHSFPIY

SEQ ID NO: 3 - DNA, 7440 bp, Mus musculus
ctaataaatagggaaactatgaggactttctccatcttccgagtgttcagaagcagcaagaggactaggcagttcaaatccaaactgttccgacagtttttttagcttctcttctaataggatattctttttcacttcttccttataattatacttcaggtcttcaatttcttcaaaaaatgaaggatcaaaattttccagttcttttttcagctttttaacttcctccttcgaatgttgcttttctagctccaactttctgagttgtgtctccaggtcatttatcttttcctttagttgatcagaatcaggtatgctactgtcagctctggtttggtccttgttaatttctatctgatggattaattctgccctttctttatccatctgattattggctaatctaagaagctggagttcccgtataagctcttgctctgtctcggcaccttcaggaacatttttgaggatctcaatctgttgttcaaggtcttcagtgtatttcttagctttctgttctctctctgttgcttctcttacaagctgtttaaggtcagtgatactttgattctttttggcaatgtcactttcaagctctttcatcttggtctcatacactcttgagaccacaattgacttccagctcttgctgtcagcaccttccagctgtggggctctactttctgcaaactgtagtctcttcccagtttcttcgagttgagctgccatcttgtcgttcaccagctctaagttgttcttagctatccgcagtttctcagaggcttctatttctttcttaagttctttccgaagccgttcattttcggcaacaattttctcagtacctttgttcttagattcaaactgcatactcaactgacgtccaaagtgagctttaagcttttctagttcagcctttaagtttctattttcttcctcaatagtagccattttttcactagtcagtattcctgatgcctttttcaattgttcattttctctttggactttttcaactactttcttcattaacccaatggttttttctagttctgggattgtcttcccacttctaccagcccctctgacctgaccaagcttccgctcaagttccagttttcctttcttaagaaattcacacatttccttcaaatctttcacttgattctttagtcttggcaaatctttatttgcttgttcaagttgaaatttcagctcgatgttttcagatgacaacttcaaattttccttctgaagttcttgttctttttgacagtgatcatctgactctatttctgaagtcaaagactgagaatatttctcctttgaaagttttttttctaaagtatgaagtttttcttgaaggtatttattttgtaaatgtaagtcttccacaacagaatctcgtggaagagcctgctgggtcctcatgtataatatgtcattttctaggtccagatttttcttttttagctcttccaactctttttcagattccaaagctcgcactcctaaaacctggtcaacagtcattcctgttgttttcagtttcttctgcaaagtaagtttctctttatcagctttggcaaaaagttcctttaaggtattcagctgctttgccaggccgtgggcttctccttccttctcctttagtctgtttcgtagtccctctactttggtttgccatttcttaccttcttcccacctaattaattcttctttactactcttttccttcaccggctttatgtctacgtcatccacctttctttccagttggctttcaagttttttaactttcttttgaagttcatcgattaaactttgcttgttatctatcaaagttttgctctgcagtccactggacagtcttttaatctgtcttctcagttcatcattttcttgatcaattccatctttctctctaaggattttattataagctttttgctttttttgcagttcattatttaattcatttaaatcatcagctagtgaattttctttgttcttacttgttttaagagcttctttcaattttaaaagattttcatttaaatcttcaatttgtgactttagctctctagtatggcgctcaacaacttgttgaacattgagatttgcctctttttgagaagttacagcgattatacgttcctcagctgctgctgtcatttccgaccgaagttccaacagggctcgactaagtgccttttgttgcttctctttcaaggctagttggctctttagcctgtctacaagattcctcattgtggttgttggagctctggagtttgcttctttctgagcctggagttcagactttaaactctgggagtccttgtgtgcttgggctagagcatgccttaagtcctctacctctgctttcactttctttacctcactggcatgagtttcttggagccgtagtttggtattttcaaactctctgacttttaactcagtgatttctttttgtttttccaaatcttttgatactttctttagtttggtcaaaagtgaggacagagagtcatcttgttctgctactgtctgctccatctcggccagacgaatgaaatgtttgttggtgggaactggagcaggagactgcttaagtaaatcctgagctgtctgtctgaatttattgagtgaattatcggcctgttgttctaatttgtgatgaagaacatgaaggtcttcctcatgcttcttaacaatttctctttgctcctctctggccttctccagaaggtgctggtatttcttcaatacttcttccttgtgatttaaccttgcctgcatgttggcaatagtttggtgggcaattttcattgtgtgatgagatttcggctccagctcttttctttctagctcagctataagtttttctcgatcagccgtggcaggcaatcgaagcctcagttcattgattactttgtctcttgacagaatattttgctctgccaaccgtaaagcagattctttttcttttagtttctcttctagtgacttgcaagttgcttgtgttttaagaattacttgaatattctccttaatttttcttagagcaatttcaagttggtttggaagaggcaagctggggtctggcattgatcctgtagagtcttcaaacttttgtgctgcactgagtatttcattttgctgatgatcaaaaatgtctaactggcgttccagctcaacttctctttgatcccaagccatctgtctttcttcatggaacttgctttgctgaacaatttcttcctctagactgttgattgtatgctcatattcagagatgatattattcaaatatttgatttcttctttacccttgactagttctctatttagcttaagttcttggaggcgaagttcttctattttcacatgccaattgattaccttctgggctcccctggcatcctttaaagtactgatcaattcttctaagccttttaattttaattccaactccagtgttttgttttccatatttctgtgttcctgttgcgaattcttcatttcttgcattatcttaagtttgtcattttgcaactgaatcatcgttttggagaacttttcctgctgtgctaagggtagagctccactgaactgtcttcgaagcgactgaatggtttggcgcaggtgttttgctctgtttctaccttccaaacgagcatagtagagcgcctgctctttttcatccagtttctgttctaagcgcaaattgtaggcttccatcttctggagtttggacgtaactgactctaacttaccgagggcagtggcctcactaatttgaagagagacaacatgttggtgcaatttggcaattagagccttttcgtcagattgtgcctggaagtccagcagctgcgttctgagggattccacttccttttccctggactgttgttgcgaattcaaaaaatcaacttgtcttttggcaatatctgaaatctctctcagcttggacacttcaactttgagctccacttcactcttctctagttctagaatccgctgtcggtcagcatcacttactgccttggtcacactatcagctaattcgtctctcaacatctgctccaccttttgtgcatccaggttgattttagtaagctcagtgaacttggtttccaattcaaaattacgttcttccatttgctttaatgaagtccttaagtgctcatacattttctgacagtgttcagccctctgcctttcatttaattccttcatctccaacacagtgattttctttgaaatagaaacaatgtcactgtttgtcattgatttcttagccttatccatgtttgagtcatttcctaacttcgtttcttgttcccaggcctgttcaatggtatggagtttttcctttgtaatctccagctctttactgatagcctccatctgttcttttagcgatgcattctcacactccaggtgttctaagttacttgttctttgaacaagcatattatctttctgcaagatgtccctgtacttagtagtcagctcattgtactgtttattggctagttctaattcagacaaagaaacactattatctataaccttctgaagagctgcaatcttgaagatggccatttccttgaatctttgcaaacttccaagtttttcagtgacttcggcctccatggctatgacgtcattcctgtgtttcccgttttcctttctcaggtgccgctccatctccactaaggtggtgtactgccggatgagggacttctcgttcacttgcagaacggtgattttcctactgttttctgagagcattttcttcatctcgttcgaatccatctgaagagcactgagcaaattgttgtactcttttactttcacagcatcctgctcagcttgatcttccagttttctcttctcctctcttatcatctcagagtctgttttccaaatatccttttcacttaggtattctttatataataaactttgttgatgacgaatcactgcaaactttctgttataatcttcaagggaatcttctaaatgttttaatttcttttctttattgtctagttcctgcaaaagatgtattaagtattcattctgagaattgatgatataggcactggatggtgctatcccatcgggtaagtctatgcctttgtatactacattggagcctgcagactgacgtagaaggtcagtttccttctcaaggtggtcaatctttaagtttgcttttaccaactgctgtgaataatttacagcctctttccgagattgcctgagttcttgccttaattcttcattccttcctgtaagttggtcaacttgggcttttagatgcaagctggcatcgaagattccttctgcattctttgattccatagcgttaaccagtctttcaagactcgggatgattaaagatgtttcacctcctttcacatcagaatccttcggcatgtccttaatagcttgcaaaatttctttcataccttcttcaagttgcttattttcttcgactaattcttttagtttactctggaatttagcaattactgtcctacttctttctaaatctttttccttttcagccaattctcttgaaagaaactcattctttgattgtgtttcattcatattattgaggctcataaaatttagttttcttccttctattttattttcatgagaaaaggtttcagataagttcaagtcgtcaatggttaatcctgaggctgcgttccttttgcctctttcttgagccatttgacgaatctttcttttcaagtcaagacgctcctcctctagactttcgatctctttcaaaagaacctggttctcagctctgtactgttgctgctttaaccgtttgctgtttctaaattcagtcaaatcaatcattgtcttgggttcaaggccagcccgctctctaagggcttcgttttcatcaaggatgtcattgatcttcatctcaagcttattgatctccttggtcaacacttccatctctccatctcttattttaatttgggctttacaattctttatttcgataacagcatcttctaagccatatactccagattcataatcttttaatctcttcagagcctcaaccaattctttgtccttctccctggcatcagcctcagccagctcagctattctctcggcctcttttgttttctcttctaaaatttgtacttttgagtgaattttcatataatgagtctgctgataaaagtttgaagtacctttgtctttttggagttcatttttcaaatcttcaataataaacgtatttttttccatttctttcgtatactgttctacttgctcagtaagcatcttaatttgactgtctcgctcctggataccctgtttcagagccatgatgttacttttgtctgcatcaagttgggcatttttaagtttccctctcagactctgtagcatttgctgatattcaatgatttcatcatctttagaagacaaaattaacttccactcttccacttttgcgttaacagccatcatgactggatcgtcctcttcatccttcgccttcagaagatccgtgagctctcgaacttgcaggcgatagtgctcattctccttcttgatctggtccatgacagcatccgactgatgcacaagcgctttcatcctgttgtactcatcagtcatcttctccatctcctgcacagactcttccaggtttttcctcatttcttggttctgaacttcaatcttctcattagcttctgttaaggtctgtatttcgtccagatattgaacaagttcatagttctttttagacaactgtgatcggtagtcactgtcttctcctctccttgacagaagtgattctttctgtgaatctatttgtttctggtagtcaataatgtcctgccgaagctgctcattctttttctttagacgtttgttctctcttcttaatttgctgttttcattttctgcctcctcatttcgaagagccaattgttcattaaccttcttttctttatccaattctttttccatatcctctaattctctatctttttgttccagctgcttctcaagttggcgaatttcgtcacgtaaaaaccgagtgtcacgtccccctgcagactgctgagccatctccagttcattttccagtttcattacttttgtctttaattgattttcaaattttgcttgttcttctccagccttttcaacttcttccaaagcgagctctacttcctgggctttcatcttcattagagactgggtaattctgaatagatgtatcatgttttcttggtcttcattttttagttcatttacttccaccttggataaagatatcaataatttatctgctaactcttcttgccgtggcaggtcatctggatcaactttgattaattctttccactttatattaggtggcat

SEQ ID NO: 4 - DNA, 2970 bp, Mus musculus
ttggcagagcaaaatattctgtcaagagacaaagtaatcaatgaactgaggcttcgattgcctgccacggctgatcgagaaaaacttatagctgagctagaaagaaaagagctggagccgaaatctcatcacacaatgaaaattgcccaccaaactattgccaacatgcaggcaaggttaaatcacaaggaagaagtattgaagaaataccagcaccttctggagaaggccagagaggagcaaagagaaattgttaagaagcatgaggaagaccttcatgttcttcatcacaaattagaacaacaggccgataattcactcaataaattcagacagacagctcaggatttacttaagcagtctcctgctccagttcccaccaacaaacatttcattcgtctggccgagatggagcagacagtagcagaacaagatgactctctgtcctcacttttgaccaaactaaagaaagtatcaaaagatttggaaaaacaaaaagaaatcactgagttaaaagtcagagagtttgaaaataccaaactacggctccaagaaactcatgccagtgaggtaaagaaagtgaaagcagaggtagaggacttaaggcatgctctagcccaagcacacaaggactcccagagtttaaagtctgaactccaggctcagaaagaagcaaactccagagctccaacaaccacaatgaggaatcttgtagacaggctaaagagccaactagccttgaaagagaagcaacaaaaggcacttagtcgagccctgttggaacttcggtcggaaatgacagcagcagctgaggaacgtataatcgctgtaacttctcaaaaagaggcaaatctcaatgttcaacaagttgttgagcgccatactagagagctaaagtcacaaattgaagatttaaatgaaaatcttttaaaattgaaagaagctcttaaaacaagtaagaacaaagaaaattcactagctgatgatttaaatgaattaaataatgaactgcaaaaaaagcaaaaagcttataataaaatccttagagagaaagatggaattgatcaagaaaatgatgaactgagaagacagattaaaagactgtccagtggactgcagagcaaaactttgatagataacaagcaaagtttaatcgatgaacttcaaaagaaagttaaaaaacttgaaagccaactggaaagaaaggtggatgacgtagacataaagccggtgaaggaaaagagtagtaaagaagaattaattaggtgggaagaaggtaagaaatggcaaaccaaagtagagggactacgaaacagactaaaggagaaggaaggagaagcccacggcctggcaaagcagctgaataccttaaaggaactttttgccaaagctgataaagagaaacttactttgcagaagaaactgaaaacaacaggaatgactgttgaccaggttttaggagtgcgagctttggaatctgaaaaagagttggaagagctaaaaaagaaaaatctggacctagaaaatgacatattatacatgaggacccagcaggctcttccacgagattctgttgtggaagacttacatttacaaaataaataccttcaagaaaaacttcatactttagaaaaaaaactttcaaaggagaaatattctcagtctttgacttcagaaatagagtcagatgatcactgtcaaaaagaacaagaacttcagaaggaaaatttgaagttgtcatctgaaaacatcgagctgaaatttcaacttgaacaagcaaataaagatttgccaagactaaagaatcaagtgaaagatttgaaggaaatgtgtgaatttcttaagaaaggaaaactggaacttgagcggaagcttggtcaggtcagaggggctggtagaagtgggaagacaatcccagaactagaaaaaaccattgggttaatgaagaaagtagttgaaaaagtccaaagagaaaatgaacaattgaaaaaggcatcaggaatactgactagtgaaaaaatggctactattgaggaagaaaatagaaacttaaaggctgaactagaaaagcttaaagctcactttggacgtcagttgagtatgcagtttgaatctaagaacaaaggtactgagaaaattgttgccgaaaatgaacggcttcggaaagaacttaagaaagaaatagaagcctctgagaaactgcggatagctaagaacaacttagagctggtgaacgacaagatggcagctcaactcgaagaaactgggaagagactacagtttgcagaaagtagagccccacagctggaaggtgctgacagcaagagctggaagtcaattgtggtctcaagagtgtatgagaccaagatgaaagagcttgaaagtgacattgccaaaaagaatcaaagtatcactgaccttaaacagcttgtaagagaagcaacagagagagaacagaaagctaagaaatacactgaagaccttgaacaacagattgagatcctcaaaaatgttcctgaaggtgccgagacagagcaagagcttatacgggaactccagcttcttagattagccaataatcagatggataaagaaagggcagaattaatccatcagatagaaattaacaaggaccaaaccagagctgacagtagcatacctgattctgatcaactaaaggaaaagataaatgacctggagacacaactcagaaagttggagctagaaaagcaacattcgaaggaggaagttaaaaagctgaaaaaagaactggaaaattttgatccttcattttttgaagaaattgaagacctgaagtataattataaggaagaagtgaaaaagaatatcctattagaagagaagctaaaaaaactgtcggaacagtttggatttgaactgcctagtcctcttgctgcttctgaacactcggaagatggagaaagtcctcatagtttccctatttattag

SEQ ID NO: 5 - protein, 989 aa, Mus musculus
LAEQNILSRDKVINELRLRLPATADREKLIAELERKELEPKSHHTMKIAHQTIANMQARLNHKEEVLKKYQHLLEKAREEQREIVKKHEEDLHVLHHKLEQQADNSLNKFRQTAQDLLKQSPAPVPTNKHFIRLAEMEQTVAEQDDSLSSLLTKLKKVSKDLEKQKEITELKVREFENTKLRLQETHASEVKKVKAEVEDLRHALAQAHKDSQSLKSELQAQKEANSRAPTTTMRNLVDRLKSQLALKEKQQKALSRALLELRSEMTAAAEERIIAVTSQKEANLNVQQVVERHTRELKSQIEDLNENLLKLKEALKTSKNKENSLADDLNELNNELQKKQKAYNKILREKDGIDQENDELRRQIKRLSSGLQSKTLIDNKQSLIDELQKKVKKLESQLERKVDDVDIKPVKEKSSKEELIRWEEGKKWQTKVEGLRNRLKEKEGEAHGLAKQLNTLKELFAKADKEKLTLQKKLKTTGMTVDQVLGVRALESEKELEELKKKNLDLENDILYMRTQQALPRDSVVEDLHLQNKYLQEKLHTLEKKLSKEKYSQSLTSEIESDDHCQKEQELQKENLKLSSENIELKFQLEQANKDLPRLKNQVKDLKEMCEFLKKGKLELERKLGQVRGAGRSGKTIPELEKTIGLMKKVVEKVQRENEQLKKASGILTSEKMATIEEENRNLKAELEKLKAHFGRQLSMQFESKNKGTEKIVAENERLRKELKKEIEASEKLRIAKNNLELVNDKMAAQLEETGKRLQFAESRAPQLEGADSKSWKSIVVSRVYETKMKELESDIAKKNQSITDLKQLVREATEREQKAKKYTEDLEQQIEILKNVPEGAETEQELIRELQLLRLANNQMDKERAELIHQIEINKDQTRADSSIPDSDQLKEKINDLETQLRKLELEKQHSKEEVKKLKKELENFDPSFFEEIEDLKYNYKEEVKKNILLEEKLKKLSEQFGFELPSPLAASEHSEDGESPHSFPIY

SEQ ID NO: 6 - DNA, 2970 bp, Mus musculus
ctaataaatagggaaactatgaggactttctccatcttccgagtgttcagaagcagcaagaggactaggcagttcaaatccaaactgttccgacagtttttttagcttctcttctaataggatattctttttcacttcttccttataattatacttcaggtcttcaatttcttcaaaaaatgaaggatcaaaattttccagttcttttttcagctttttaacttcctccttcgaatgttgcttttctagctccaactttctgagttgtgtctccaggtcatttatcttttcctttagttgatcagaatcaggtatgctactgtcagctctggtttggtccttgttaatttctatctgatggattaattctgccctttctttatccatctgattattggctaatctaagaagctggagttcccgtataagctcttgctctgtctcggcaccttcaggaacatttttgaggatctcaatctgttgttcaaggtcttcagtgtatttcttagctttctgttctctctctgttgcttctcttacaagctgtttaaggtcagtgatactttgattctttttggcaatgtcactttcaagctctttcatcttggtctcatacactcttgagaccacaattgacttccagctcttgctgtcagcaccttccagctgtggggctctactttctgcaaactgtagtctcttcccagtttcttcgagttgagctgccatcttgtcgttcaccagctctaagttgttcttagctatccgcagtttctcagaggcttctatttctttcttaagttctttccgaagccgttcattttcggcaacaattttctcagtacctttgttcttagattcaaactgcatactcaactgacgtccaaagtgagctttaagcttttctagttcagcctttaagtttctattttcttcctcaatagtagccattttttcactagtcagtattcctgatgcctttttcaattgttcattttctctttggactttttcaactactttcttcattaacccaatggttttttctagttctgggattgtcttcccacttctaccagcccctctgacctgaccaagcttccgctcaagttccagttttcctttcttaagaaattcacacatttccttcaaatctttcacttgattctttagtcttggcaaatctttatttgcttgttcaagttgaaatttcagctcgatgttttcagatgacaacttcaaattttccttctgaagttcttgttctttttgacagtgatcatctgactctatttctgaagtcaaagactgagaatatttctcctttgaaagttttttttctaaagtatgaagtttttcttgaaggtatttattttgtaaatgtaagtcttccacaacagaatctcgtggaagagcctgctgggtcctcatgtataatatgtcattttctaggtccagatttttcttttttagctcttccaactctttttcagattccaaagctcgcactcctaaaacctggtcaacagtcattcctgttgttttcagtttcttctgcaaagtaagtttctctttatcagctttggcaaaaagttcctttaaggtattcagctgctttgccaggccgtgggcttctccttccttctcctttagtctgtttcgtagtccctctactttggtttgccatttcttaccttcttcccacctaattaattcttctttactactcttttccttcaccggctttatgtctacgtcatccacctttctttccagttggctttcaagttttttaactttcttttgaagttcatcgattaaactttgcttgttatctatcaaagttttgctctgcagtccactggacagtcttttaatctgtcttctcagttcatcattttcttgatcaattccatctttctctctaaggattttattataagctttttgctttttttgcagttcattatttaattcatttaaatcatcagctagtgaattttctttgttcttacttgttttaagagcttctttcaattttaaaagattttcatttaaatcttcaatttgtgactttagctctctagtatggcgctcaacaacttgttgaacattgagatttgcctctttttgagaagttacagcgattatacgttcctcagctgctgctgtcatttccgaccgaagttccaacagggctcgactaagtgccttttgttgcttctctttcaaggctagttggctctttagcctgtctacaagattcctcattgtggttgttggagctctggagtttgcttctttctgagcctggagttcagactttaaactctgggagtccttgtgtgcttgggctagagcatgccttaagtcctctacctctgctttcactttctttacctcactggcatgagtttcttggagccgtagtttggtattttcaaactctctgacttttaactcagtgatttctttttgtttttccaaatcttttgatactttctttagtttggtcaaaagtgaggacagagagtcatcttgttctgctactgtctgctccatctcggccagacgaatgaaatgtttgttggtgggaactggagcaggagactgcttaagtaaatcctgagctgtctgtctgaatttattgagtgaattatcggcctgttgttctaatttgtgatgaagaacatgaaggtcttcctcatgcttcttaacaatttctctttgctcctctctggccttctccagaaggtgctggtatttcttcaatacttcttccttgtgatttaaccttgcctgcatgttggcaatagtttggtgggcaattttcattgtgtgatgagatttcggctccagctcttttctttctagctcagctataagtttttctcgatcagccgtggcaggcaatcgaagcctcagttcattgattactttgtctcttgacagaatattttgctctgccaa

SEQ ID NO: 7 - DNA, 7440 bp, Homo sapiens
atgccacctaatataaactggaaagaaataatgaaagttgacccagatgacctgccccgtcaagaagaactggcagataatttattgatttccttatccaaggtggaagtaaatgagctaaaaagtgaaaagcaagaaaatgtgatacaccttttcagaattactcagtcactaatgaagatgaaagctcaagaagtggagctggctttggaagaagtagaaaaagctggagaagaacaagcaaaatttgaaaatcaattaaaaactaaagtaatgaaactggaaaatgaactggagatggctcagcagtctgcaggtggacgagatactcggtttttacgtaatgaaatttgccaacttgaaaaacaattagaacaaaaagatagagaattggaggacatggaaaaggagttggagaaagagaagaaagttaatgagcaattggctcttcgaaatgaggaggcagaaaatgaaaacagcaaattaagaagagagaacaaacgtctaaagaaaaagaatgaacaactttgtcaggatattattgactaccagaaacaaatagattcacagaaagaaacacttttatcaagaagaggggaagacagtgactaccgatcacagttgtctaaaaaaaactatgagcttatccaatatcttgatgaaattcagactttaacagaagctaatgagaaaattgaagttcagaatcaagaaatgagaaaaaatttagaagagtctgtacaggaaatggagaagatgactgatgaatataatagaatgaaagctattgtgcatcagacagataatgtaatagatcagttaaaaaaagaaaacgatcattatcaacttcaagtgcaggagcttacagatcttctgaaatcaaaaaatgaagaagatgatccaattatggtagctgtcaatgcaaaagtagaagaatggaagctaattttgtcttctaaagatgatgaaattattgagtatcagcaaatgttacataacctaagggagaaacttaagaatgctcagcttgatgctgataaaagtaatgttatggctctacagcagggtatacaggaacgagacagtcaaattaagatgctcaccgaacaagtagaacaatatacaaaagaaatggaaaagaatacttgtattattgaagatttgaaaaatgagctccaaagaaacaaaggtgcttcaaccctttctcaacagactcatatgaaaattcagtcaacgttagacattttaaaagagaaaactaaagaggctgagagaacagctgaactggctgaggctgatgctagggaaaaggataaagaattagttgaggctctgaagaggttaaaagattatgaatcgggagtatatggtttagaagatgctgtcgttgaaataaagaattgtaaaaaccaaattaaaataagagatcgagagattgaaatattaacaaaggaaatcaataaacttgaattgaagatcagtgatttccttgatgaaaatgaggcacttagagagcgtgtgggccttgaaccaaagacaatgattgatttaactgaatttagaaatagcaaacacttaaaacagcagcagtacagagctgaaaaccagattcttttgaaagagattgaaagtctagaggaagaacgacttgatctgaaaaaaaaaattcgtcaaatggctcaagaaagaggaaaaagaagtgcaacttcaggattaaccactgaggacctgaacctaactgaaaacatttctcaaggagatagaataagtgaaagaaaattggatttattgagcctcaaaaatatgagtgaagcacaatcaaagaatgaatttctttcaagagaactaattgaaaaagaaagagatttagaaaggagtaggacagtgatagccaaatttcagaataaattaaaagaattagttgaagaaaataagcaacttgaagaaggtatgaaagaaatattgcaagcaattaaggaaatgcagaaagatcctgatgttaaaggaggagaaacatctctaattatccctagccttgaaagactagttaatgctatagaatcaaagaatgcagaaggaatctttgatgcgagtctgcatttgaaagcccaagttgatcagcttaccggaagaaatgaagaattaagacaggagctcagggaatctcggaaagaggctataaattattcacagcagttggcaaaagctaatttaaagatagaccatcttgaaaaagaaactagtcttttacgacaatcagaaggatcgaatgttgtttttaaaggaattgacttacctgatgggatagcaccatctagtgccagtatcattaattctcagaatgaatatttaatacatttgttacaggaactagaaaataaagaaaaaaagttaaagaatttagaagattctcttgaagattacaacagaaaatttgctgtaattcgtcatcaacaaagtttgttgtataaagaatacctaagtgaaaaggagacctggaaaacagaatctaaaacaataaaagaggaaaagagaaaacttgaggatcaagtccaacaagatgctataaaagtaaaagaatataataatttgctcaatgctcttcagatggattcggatgaaatgaaaaaaatacttgcagaaaatagtaggaaaattactgttttgcaagtgaatgaaaaatcacttataaggcaatatacaaccttagtagaattggagcgacaacttagaaaagaaaatgagaagcaaaagaatgaattgttgtcaatggaggctgaagtttgtgaaaaaattgggtgtttgcaaagatttaaggaaatggccattttcaagattgcagctctccaaaaagttgtagataatagtgtttctttgtctgaactagaactggctaataaacagtacaatgaactgactgctaagtacagggacatcttgcaaaaagataatatgcttgttcaaagaacaagtaacttggaacacctggagtgtgaaaacatctccttaaaagaacaagtggagtctataaataaagaactggagattaccaaggaaaaacttcacactattgaacaagcctgggaacaggaaactaaattaggtaatgaatctagcatggataaggcaaagaaatcaataaccaacagtgacattgtttccatttcaaaaaaaataactatgctggaaatgaaggaattaaatgaaaggcagcgggctgaacattgtcaaaaaatgtatgaacacttacggacttcgttaaagcaaatggaggaacgtaattttgaattggaaaccaaatttgctgagcttaccaaaatcaatttggatgcacagaaggtggaacagatgttaagagatgaattagctgatagtgtgagcaaggcagtaagtgatgctgataggcaacggattctagaattagagaagaatgaaatggaactaaaagttgaagtgtcaaaactgagagagatttctgatattgccagaagacaagttgaaattttgaatgcacaacaacaatctagggacaaggaagtagagtccctcagaatgcaactgctagactatcaggcacagtctgatgaaaagtcgctcattgccaagttgcaccaacataatgtctctcttcaactgagtgaggctactgctcttggtaagttggagtcaattacatctaaactgcagaagatggaggcctacaacttgcgcttagagcagaaacttgatgaaaaagaacaggctctctattatgctcgtttggagggaagaaacagagcaaaacatctgcgccaaacaattcagtctctacgacgacagtttagtggagctttacccttggcacaacaggaaaagttctccaaaacaatgattcaactacaaaatgacaaacttaagataatgcaagaaatgaaaaattctcaacaagaacatagaaatatggagaacaaaacattggagatggaattaaaattaaagggcctggaagagttaataagcactttaaaggataccaaaggagcccaaaaggtaatcaactggcatatgaaaatagaagaacttcgtcttcaagaacttaaactaaatcgggaattagtcaaggataaagaagaaataaaatatttgaataacataatttctgaatatgaacgtacaatcagcagtcttgaagaagaaattgtgcaacagaacaagtttcatgaagaaagacaaatggcctgggatcaaagagaagttgacctggaacgccaactagacatttttgaccgtcagcaaaatgaaatactaaatgcggcacaaaagtttgaagaagctacaggatcaatccctgaccctagtttgccccttccaaatcaacttgagatcgctctaaggaaaattaaggagaacattcgaataattctagaaacacgggcaacttgcaaatcactagaagagaaactaaaagagaaagaatctgctttaaggttagcagaacaaaatatactgtcaagagacaaagtaatcaatgaactgaggcttcgattgcctgccactgcagaaagagaaaagctcatagctgagctaggcagaaaagagatggaaccaaaatctcaccacacattgaaaattgctcatcaaaccattgcaaacatgcaagcaaggttaaatcaaaaagaagaagtattaaagaagtatcaacgtcttctagaaaaagccagagaggagcaaagagaaattgtgaagaaacatgaggaagaccttcatattcttcatcacagattagaactacaggctgatagttcactaaataaattcaaacaaacggcttgggatttaatgaaacagtctcccactccagttcctaccaacaagcattttattcgtctggctgagatggaacagacagtagcagaacaagatgactctctttcctcactcttggtcaaactaaagaaagtatcacaagatttggagagacaaagagaaatcactgaattaaaagtaaaagaatttgaaaatatcaaattacagcttcaagaaaaccatgaagatgaagtgaaaaaagtaaaagcggaagtagaggatttaaagtatcttctggaccagtcacaaaaggagtcacagtgtttaaaatctgaacttcaggctcaaaaagaagcaaattcaagagctccaacaactacaatgagaaatctagtagaacggctaaagagccaattagccttgaaggagaaacaacagaaagcacttagtcgggcacttttagaactccgggcagaaatgacagcagctgctgaagaacgtattatttctgcaacttctcaaaaagaggcccatctcaatgttcaacaaatcgttgatcgacatactagagagctaaagacacaagttgaagatttaaatgaaaatcttttaaaattgaaagaagcacttaaaacaagtaaaaacagagaaaactcactaactgataatttgaatgacttaaataatgaactgcaaaagaaacaaaaagcctataataaaatacttagagagaaagaggaaattgatcaagagaatgatgaactgaaaaggcaaattaaaagactaaccagtggattacagggcaaacccctgacagataataaacaaagtctaattgaagaactccaaaggaaagttaaaaaactagagaaccaattagagggaaaggtggaggaagtagacctaaaacctatgaaagaaaagaatgctaaagaagaattaattaggtgggaagaaggtaaaaagtggcaagccaaaatagaaggaattcgaaacaagttaaaagagaaagagggggaagtctttactttaacaaagcagttgaatactttgaaggatctttttgccaaagccgataaagagaaacttactttgcagaggaaactaaaaacaactggcatgactgttgatcaggttttgggaatacgagctttggagtcagaaaaagaattggaagaattaaaaaagagaaatcttgacttagaaaatgatatattgtatatgagggcccaccaagctcttcctcgagattctgttgtagaagatttacatttacaaaatagatacctccaagaaaaacttcatgctttagaaaaacagttttcaaaggatacatattctaagccttcaatttcaggaatagagtcagatgatcattgtcagagagaacaggagcttcagaaggaaaacttgaagttgtcatctgaaaatattgaactgaaatttcagcttgaacaagcaaataaagatttgccaagattaaagaatcaagtcagagatttgaaggaaatgtgtgaatttcttaagaaagaaaaagcagaagttcagcggaaacttggccatgttagagggtctggtagaagtggaaagacaatcccagaactggaaaaaaccattggtttaatgaaaaaagtagttgaaaaagtccagagagaaaatgaacagttgaaaaaagcatcaggaatattgactagtgaaaaaatggctaatattgagcaggaaaatgaaaaattgaaggctgaattagaaaaacttaaagctcatcttgggcatcagttgagcatgcactatgaatccaagaccaaaggcacagaaaaaattattgctgaaaatgaaaggcttcgtaaagaacttaaaaaagaaactgatgctgcagagaaattacggatagcaaagaataatttagagatattaaatgagaagatgacagttcaactagaagagactggtaagagattgcagtttgcagaaagcagaggtccacagcttgaaggtgctgacagtaagagctggaaatccattgtggttacaagaatgtatgaaaccaagttaaaagaattggaaactgatattgccaaaaaaaatcaaagcattactgaccttaaacagcttgtaaaagaagcaacagagagagaacaaaaagttaacaaatacaatgaagaccttgaacaacagattaagattcttaaacatgttcctgaaggtgctgagacagagcaaggccttaaacgggagcttcaagttcttagattagctaatcatcagctggataaagagaaagcagaattaatccatcagatagaagctaacaaggaccaaagtggagctgaaagcaccatacctgatgctgatcaactaaaggaaaaaataaaagatctagagacacagctcaaaatgtcagatctagaaaagcagcatttgaaggaggaaataaagaagctgaaaaaagaactggaaaattttgatccttcattttttgaagaaattgaagatcttaagtataattacaaggaagaagtgaagaagaatattctcttagaagagaaggtaaaaaaactttcagaacaattgggagttgaattaactagccctgttgctgcttctgaagagtttgaagatgaagaagaaagtcctgttaatttccccatttactaa

SEQ ID NO: 8 - protein, 2479 aa, Homo sapiens
MPPNINWKEIMKVDPDDLPRQEELADNLLISLSKVEVNELKSEKQENVIHLFRITQSLMKMKAQEVELALEEVEKAGEEQAKFENQLKTKVMKLENELEMAQQSAGGRDTRFLRNEICQLEKQLEQKDRELEDMEKELEKEKKVNEQLALRNEEAENENSKLRRENKRLKKKNEQLCQDIIDYQKQIDSQKETLLSRRGEDSDYRSQLSKKNYELIQYLDEIQTLTEANEKIEVQNQEMRKNLEESVQEMEKMTDEYNRMKAIVHQTDNVIDQLKKENDHYQLQVQELTDLLKSKNEEDDPIMVAVNAKVEEWKLILSSKDDEIIEYQQMLHNLREKLKNAQLDADKSNVMALQQGIQERDSQIKMLTEQVEQYTKEMEKNTCIIEDLKNELQRNKGASTLSQQTHMKIQSTLDILKEKTKEAERTAELAEADAREKDKELVEALKRLKDYESGVYGLEDAVVEIKNCKNQIKIRDREIEILTKEINKLELKISDFLDENEALRERVGLEPKTMIDLTEFRNSKHLKQQQYRAENQILLKEIESLEEERLDLKKKIRQMAQERGKRSATSGLTTEDLNLTENISQGDRISERKLDLLSLKNMSEAQSKNEFLSRELIEKERDLERSRTVIAKFQNKLKELVEENKQLEEGMKEILQAIKEMQKDPDVKGGETSLIIPSLERLVNAIESKNAEGIFDASLHLKAQVDQLTGRNEELRQELRESRKEAINYSQQLAKANLKIDHLEKETSLLRQSEGSNVVFKGIDLPDGIAPSSASIINSQNEYLIHLLQELENKEKKLKNLEDSLEDYNRKFAVIRHQQSLLYKEYLSEKETWKTESKTIKEEKRKLEDQVQQDAIKVKEYNNLLNALQMDSDEMKKILAENSRKITVLQVNEKSLIRQYTTLVELERQLRKENEKQKNELLSMEAEVCEKIGCLQRFKEMAIFKIAALQKVVDNSVSLSELELANKQYNELTAKYRDILQKDNMLVQRTSNLEHLECENISLKEQVESINKELEITKEKLHTIEQAWEQETKLGNESSMDKAKKSITNSDIVSISKKITMLEMKELNERQRAEHCQKMYEHLRTSLKQMEERNFELETKFAELTKINLDAQKVEQMLRDELADSVSKAVSDADRQRILELEKNEMELKVEVSKLREISDIARRQVEILNAQQQSRDKEVESLRMQLLDYQAQSDEKSLIAKLHQHNVSLQLSEATALGKLESITSKLQKMEAYNLRLEQKLDEKEQALYYARLEGRNRAKHLRQTIQSLRRQFSGALPLAQQEKFSKTMIQLQNDKLKIMQEMKNSQQEHRNMENKTLEMELKLKGLEELISTLKDTKGAQKVINWHMKIEELRLQELKLNRELVKDKEEIKYLNNIISEYERTISSLEEEIVQQNKFHEERQMAWDQREVDLERQLDIFDRQQNEILNAAQKFEEATGSIPDPSLPLPNQLEIALRKIKENIRIILETRATCKSLEEKLKEKESALRLAEQNILSRDKVINELRLRLPATAEREKLIAELGRKEMEPKSHHTLKIAHQTIANMQARLNQKEEVLKKYQRLLEKAREEQREIVKKHEEDLHILHHRLELQADSSLNKFKQTAWDLMKQSPTPVPTNKHFIRLAEMEQTVAEQDDSLSSLLVKLKKVSQDLERQREITELKVKEFENIKLQLQENHEDEVKKVKAEVEDLKYLLDQSQKESQCLKSELQAQKEANSRAPTTTMRNLVERLKSQLALKEKQQKALSRALLELRAEMTAAAEERIISATSQKEAHLNVQQIVDRHTRELKTQVEDLNENLLKLKEALKTSKNRENSLTDNLNDLNNELQKKQKAYNKILREKEEIDQENDELKRQIKRLTSGLQGKPLTDNKQSLIEELQRKVKKLENQLEGKVEEVDLKPMKEKNAKEELIRWEEGKKWQAKIEGIRNKLKEKEGEVFTLTKQLNTLKDLFAKADKEKLTLQRKLKTTGMTVDQVLGIRALESEKELEELKKRNLDLENDILYMRAHQALPRDSVVEDLHLQNRYLQEKLHALEKQFSKDTYSKPSISGIESDDHCQREQELQKENLKLSSENIELKFQLEQANKDLPRLKNQVRDLKEMCEFLKKEKAEVQRKLGHVRGSGRSGKTIPELEKTIGLMKKVVEKVQRENEQLKKASGILTSEKMANIEQENEKLKAELEKLKAHLGHQLSMHYESKTKGTEKIIAENERLRKELKKETDAAEKLRIAKNNLEILNEKMTVQLEETGKRLQFAESRGPQLEGADSKSWKSIVVTRMYETKLKELETDIAKKNQSITDLKQLVKEATEREQKVNKYNEDLEQQIKILKHVPEGAETEQGLKRELQVLRLANHQLDKEKAELIHQIEANKDQSGAESTIPDADQLKEKIKDLETQLKMSDLEKQHLKEEIKKLKKELENFDPSFFEEIEDLKYNYKEEVKKNILLEEKVKKLSEQLGVELTSPVAASEEFEDEEESPVNFPIY

SEQ ID NO: 9 - DNA, 7440 bp, Homo sapiens
ttagtaaatggggaaattaacaggactttcttcttcatcttcaaactcttcagaagcagcaacagggctagttaattcaactcccaattgttctgaaagtttttttaccttctcttctaagagaatattcttcttcacttcttccttgtaattatacttaagatcttcaatttcttcaaaaaatgaaggatcaaaattttccagttcttttttcagcttctttatttcctccttcaaatgctgcttttctagatctgacattttgagctgtgtctctagatcttttattttttcctttagttgatcagcatcaggtatggtgctttcagctccactttggtccttgttagcttctatctgatggattaattctgctttctctttatccagctgatgattagctaatctaagaacttgaagctcccgtttaaggccttgctctgtctcagcaccttcaggaacatgtttaagaatcttaatctgttgttcaaggtcttcattgtatttgttaactttttgttctctctctgttgcttcttttacaagctgtttaaggtcagtaatgctttgattttttttggcaatatcagtttccaattcttttaacttggtttcatacattcttgtaaccacaatggatttccagctcttactgtcagcaccttcaagctgtggacctctgctttctgcaaactgcaatctcttaccagtctcttctagttgaactgtcatcttctcatttaatatctctaaattattctttgctatccgtaatttctctgcagcatcagtttcttttttaagttctttacgaagcctttcattttcagcaataattttttctgtgcctttggtcttggattcatagtgcatgctcaactgatgcccaagatgagctttaagtttttctaattcagccttcaatttttcattttcctgctcaatattagccattttttcactagtcaatattcctgatgcttttttcaactgttcattttctctctggactttttcaactacttttttcattaaaccaatggttttttccagttctgggattgtctttccacttctaccagaccctctaacatggccaagtttccgctgaacttctgctttttctttcttaagaaattcacacatttccttcaaatctctgacttgattctttaatcttggcaaatctttatttgcttgttcaagctgaaatttcagttcaatattttcagatgacaacttcaagttttccttctgaagctcctgttctctctgacaatgatcatctgactctattcctgaaattgaaggcttagaatatgtatcctttgaaaactgtttttctaaagcatgaagtttttcttggaggtatctattttgtaaatgtaaatcttctacaacagaatctcgaggaagagcttggtgggccctcatatacaatatatcattttctaagtcaagatttctcttttttaattcttccaattctttttctgactccaaagctcgtattcccaaaacctgatcaacagtcatgccagttgtttttagtttcctctgcaaagtaagtttctctttatcggctttggcaaaaagatccttcaaagtattcaactgctttgttaaagtaaagacttccccctctttctcttttaacttgtttcgaattccttctattttggcttgccactttttaccttcttcccacctaattaattcttctttagcattcttttctttcataggttttaggtctacttcctccacctttccctctaattggttctctagttttttaactttcctttggagttcttcaattagactttgtttattatctgtcaggggtttgccctgtaatccactggttagtcttttaatttgccttttcagttcatcattctcttgatcaatttcctctttctctctaagtattttattataggctttttgtttcttttgcagttcattatttaagtcattcaaattatcagttagtgagttttctctgtttttacttgttttaagtgcttctttcaattttaaaagattttcatttaaatcttcaacttgtgtctttagctctctagtatgtcgatcaacgatttgttgaacattgagatgggcctctttttgagaagttgcagaaataatacgttcttcagcagctgctgtcatttctgcccggagttctaaaagtgcccgactaagtgctttctgttgtttctccttcaaggctaattggctctttagccgttctactagatttctcattgtagttgttggagctcttgaatttgcttctttttgagcctgaagttcagattttaaacactgtgactccttttgtgactggtccagaagatactttaaatcctctacttccgcttttacttttttcacttcatcttcatggttttcttgaagctgtaatttgatattttcaaattcttttacttttaattcagtgatttctctttgtctctccaaatcttgtgatactttctttagtttgaccaagagtgaggaaagagagtcatcttgttctgctactgtctgttccatctcagccagacgaataaaatgcttgttggtaggaactggagtgggagactgtttcattaaatcccaagccgtttgtttgaatttatttagtgaactatcagcctgtagttctaatctgtgatgaagaatatgaaggtcttcctcatgtttcttcacaatttctctttgctcctctctggctttttctagaagacgttgatacttctttaatacttcttctttttgatttaaccttgcttgcatgtttgcaatggtttgatgagcaattttcaatgtgtggtgagattttggttccatctcttttctgcctagctcagctatgagcttttctctttctgcagtggcaggcaatcgaagcctcagttcattgattactttgtctcttgacagtatattttgttctgctaaccttaaagcagattctttctcttttagtttctcttctagtgatttgcaagttgcccgtgtttctagaattattcgaatgttctccttaattttccttagagcgatctcaagttgatttggaaggggcaaactagggtcagggattgatcctgtagcttcttcaaacttttgtgccgcatttagtatttcattttgctgacggtcaaaaatgtctagttggcgttccaggtcaacttctctttgatcccaggccatttgtctttcttcatgaaacttgttctgttgcacaatttcttcttcaagactgctgattgtacgttcatattcagaaattatgttattcaaatattttatttcttctttatccttgactaattcccgatttagtttaagttcttgaagacgaagttcttctattttcatatgccagttgattaccttttgggctcctttggtatcctttaaagtgcttattaactcttccaggccctttaattttaattccatctccaatgttttgttctccatatttctatgttcttgttgagaatttttcatttcttgcattatcttaagtttgtcattttgtagttgaatcattgttttggagaacttttcctgttgtgccaagggtaaagctccactaaactgtcgtcgtagagactgaattgtttggcgcagatgttttgctctgtttcttccctccaaacgagcataatagagagcctgttctttttcatcaagtttctgctctaagcgcaagttgtaggcctccatcttctgcagtttagatgtaattgactccaacttaccaagagcagtagcctcactcagttgaagagagacattatgttggtgcaacttggcaatgagcgacttttcatcagactgtgcctgatagtctagcagttgcattctgagggactctacttccttgtccctagattgttgttgtgcattcaaaatttcaacttgtcttctggcaatatcagaaatctctctcagttttgacacttcaacttttagttccatttcattcttctctaattctagaatccgttgcctatcagcatcacttactgccttgctcacactatcagctaattcatctcttaacatctgttccaccttctgtgcatccaaattgattttggtaagctcagcaaatttggtttccaattcaaaattacgttcctccatttgctttaacgaagtccgtaagtgttcatacattttttgacaatgttcagcccgctgcctttcatttaattccttcatttccagcatagttattttttttgaaatggaaacaatgtcactgttggttattgatttctttgccttatccatgctagattcattacctaatttagtttcctgttcccaggcttgttcaatagtgtgaagtttttccttggtaatctccagttctttatttatagactccacttgttcttttaaggagatgttttcacactccaggtgttccaagttacttgttctttgaacaagcatattatctttttgcaagatgtccctgtacttagcagtcagttcattgtactgtttattagccagttctagttcagacaaagaaacactattatctacaactttttggagagctgcaatcttgaaaatggccatttccttaaatctttgcaaacacccaattttttcacaaacttcagcctccattgacaacaattcattcttttgcttctcattttcttttctaagttgtcgctccaattctactaaggttgtatattgccttataagtgatttttcattcacttgcaaaacagtaattttcctactattttctgcaagtatttttttcatttcatccgaatccatctgaagagcattgagcaaattattatattcttttacttttatagcatcttgttggacttgatcctcaagttttctcttttcctcttttattgttttagattctgttttccaggtctccttttcacttaggtattctttatacaacaaactttgttgatgacgaattacagcaaattttctgttgtaatcttcaagagaatcttctaaattctttaactttttttctttattttctagttcctgtaacaaatgtattaaatattcattctgagaattaatgatactggcactagatggtgctatcccatcaggtaagtcaattcctttaaaaacaacattcgatccttctgattgtcgtaaaagactagtttctttttcaagatggtctatctttaaattagcttttgccaactgctgtgaataatttatagcctctttccgagattccctgagctcctgtcttaattcttcatttcttccggtaagctgatcaacttgggctttcaaatgcagactcgcatcaaagattccttctgcattctttgattctatagcattaactagtctttcaaggctagggataattagagatgtttctcctcctttaacatcaggatctttctgcatttccttaattgcttgcaatatttctttcataccttcttcaagttgcttattttcttcaactaattcttttaatttattctgaaatttggctatcactgtcctactcctttctaaatctctttctttttcaattagttctcttgaaagaaattcattctttgattgtgcttcactcatatttttgaggctcaataaatccaattttctttcacttattctatctccttgagaaatgttttcagttaggttcaggtcctcagtggttaatcctgaagttgcacttctttttcctctttcttgagccatttgacgaattttttttttcagatcaagtcgttcttcctctagactttcaatctctttcaaaagaatctggttttcagctctgtactgctgctgttttaagtgtttgctatttctaaattcagttaaatcaatcattgtctttggttcaaggcccacacgctctctaagtgcctcattttcatcaaggaaatcactgatcttcaattcaagtttattgatttcctttgttaatatttcaatctctcgatctcttattttaatttggtttttacaattctttatttcaacgacagcatcttctaaaccatatactcccgattcataatcttttaacctcttcagagcctcaactaattctttatccttttccctagcatcagcctcagccagttcagctgttctctcagcctctttagttttctcttttaaaatgtctaacgttgactgaattttcatatgagtctgttgagaaagggttgaagcacctttgtttctttggagctcatttttcaaatcttcaataatacaagtattcttttccatttcttttgtatattgttctacttgttcggtgagcatcttaatttgactgtctcgttcctgtataccctgctgtagagccataacattacttttatcagcatcaagctgagcattcttaagtttctcccttaggttatgtaacatttgctgatactcaataatttcatcatctttagaagacaaaattagcttccattcttctacttttgcattgacagctaccataattggatcatcttcttcattttttgatttcagaagatctgtaagctcctgcacttgaagttgataatgatcgttttctttttttaactgatctattacattatctgtctgatgcacaatagctttcattctattatattcatcagtcatcttctccatttcctgtacagactcttctaaattttttctcatttcttgattctgaacttcaattttctcattagcttctgttaaagtctgaatttcatcaagatattggataagctcatagttttttttagacaactgtgatcggtagtcactgtcttcccctcttcttgataaaagtgtttctttctgtgaatctatttgtttctggtagtcaataatatcctgacaaagttgttcattctttttctttagacgtttgttctctcttcttaatttgctgttttcattttctgcctcctcatttcgaagagccaattgctcattaactttcttctctttctccaactccttttccatgtcctccaattctctatctttttgttctaattgtttttcaagttggcaaatttcattacgtaaaaaccgagtatctcgtccacctgcagactgctgagccatctccagttcattttccagtttcattactttagtttttaattgattttcaaattttgcttgttcttctccagctttttctacttcttccaaagccagctccacttcttgagctttcatcttcattagtgactgagtaattctgaaaaggtgtatcacattttcttgcttttcactttttagctcatttacttccaccttggataaggaaatcaataaattatctgccagttcttcttgacggggcaggtcatctgggtcaactttcattatttctttccagtttatattaggtggcat

SEQ ID NO: 10 - DNA, 2973 bp, Homo sapiens
ttagcagaacaaaatatactgtcaagagacaaagtaatcaatgaactgaggcttcgattgcctgccactgcagaaagagaaaagctcatagctgagctaggcagaaaagagatggaaccaaaatctcaccacacattgaaaattgctcatcaaaccattgcaaacatgcaagcaaggttaaatcaaaaagaagaagtattaaagaagtatcaacgtcttctagaaaaagccagagaggagcaaagagaaattgtgaagaaacatgaggaagaccttcatattcttcatcacagattagaactacaggctgatagttcactaaataaattcaaacaaacggcttgggatttaatgaaacagtctcccactccagttcctaccaacaagcattttattcgtctggctgagatggaacagacagtagcagaacaagatgactctctttcctcactcttggtcaaactaaagaaagtatcacaagatttggagagacaaagagaaatcactgaattaaaagtaaaagaatttgaaaatatcaaattacagcttcaagaaaaccatgaagatgaagtgaaaaaagtaaaagcggaagtagaggatttaaagtatcttctggaccagtcacaaaaggagtcacagtgtttaaaatctgaacttcaggctcaaaaagaagcaaattcaagagctccaacaactacaatgagaaatctagtagaacggctaaagagccaattagccttgaaggagaaacaacagaaagcacttagtcgggcacttttagaactccgggcagaaatgacagcagctgctgaagaacgtattatttctgcaacttctcaaaaagaggcccatctcaatgttcaacaaatcgttgatcgacatactagagagctaaagacacaagttgaagatttaaatgaaaatcttttaaaattgaaagaagcacttaaaacaagtaaaaacagagaaaactcactaactgataatttgaatgacttaaataatgaactgcaaaagaaacaaaaagcctataataaaatacttagagagaaagaggaaattgatcaagagaatgatgaactgaaaaggcaaattaaaagactaaccagtggattacagggcaaacccctgacagataataaacaaagtctaattgaagaactccaaaggaaagttaaaaaactagagaaccaattagagggaaaggtggaggaagtagacctaaaacctatgaaagaaaagaatgctaaagaagaattaattaggtgggaagaaggtaaaaagtggcaagccaaaatagaaggaattcgaaacaagttaaaagagaaagagggggaagtctttactttaacaaagcagttgaatactttgaaggatctttttgccaaagccgataaagagaaacttactttgcagaggaaactaaaaacaactggcatgactgttgatcaggttttgggaatacgagctttggagtcagaaaaagaattggaagaattaaaaaagagaaatcttgacttagaaaatgatatattgtatatgagggcccaccaagctcttcctcgagattctgttgtagaagatttacatttacaaaatagatacctccaagaaaaacttcatgctttagaaaaacagttttcaaaggatacatattctaagccttcaatttcaggaatagagtcagatgatcattgtcagagagaacaggagcttcagaaggaaaacttgaagttgtcatctgaaaatattgaactgaaatttcagcttgaacaagcaaataaagatttgccaagattaaagaatcaagtcagagatttgaaggaaatgtgtgaatttcttaagaaagaaaaagcagaagttcagcggaaacttggccatgttagagggtctggtagaagtggaaagacaatcccagaactggaaaaaaccattggtttaatgaaaaaagtagttgaaaaagtccagagagaaaatgaacagttgaaaaaagcatcaggaatattgactagtgaaaaaatggctaatattgagcaggaaaatgaaaaattgaaggctgaattagaaaaacttaaagctcatcttgggcatcagttgagcatgcactatgaatccaagaccaaaggcacagaaaaaattattgctgaaaatgaaaggcttcgtaaagaacttaaaaaagaaactgatgctgcagagaaattacggatagcaaagaataatttagagatattaaatgagaagatgacagttcaactagaagagactggtaagagattgcagtttgcagaaagcagaggtccacagcttgaaggtgctgacagtaagagctggaaatccattgtggttacaagaatgtatgaaaccaagttaaaagaattggaaactgatattgccaaaaaaaatcaaagcattactgaccttaaacagcttgtaaaagaagcaacagagagagaacaaaaagttaacaaatacaatgaagaccttgaacaacagattaagattcttaaacatgttcctgaaggtgctgagacagagcaaggccttaaacgggagcttcaagttcttagattagctaatcatcagctggataaagagaaagcagaattaatccatcagatagaagctaacaaggaccaaagtggagctgaaagcaccatacctgatgctgatcaactaaaggaaaaaataaaagatctagagacacagctcaaaatgtcagatctagaaaagcagcatttgaaggaggaaataaagaagctgaaaaaagaactggaaaattttgatccttcattttttgaagaaattgaagatcttaagtataattacaaggaagaagtgaagaagaatattctcttagaagagaaggtaaaaaaactttcagaacaattgggagttgaattaactagccctgttgctgcttctgaagagtttgaagatgaagaagaaagtcctgttaatttccccatttactaa

SEQ ID NO: 11 - protein, 990 aa, Homo sapiens
LAEQNILSRDKVINELRLRLPATAEREKLIAELGRKEMEPKSHHTLKIAHQTIANMQARLNQKEEVLKKYQRLLEKAREEQREIVKKHEEDLHILHHRLELQADSSLNKFKQTAWDLMKQSPTPVPTNKHFIRLAEMEQTVAEQDDSLSSLLVKLKKVSQDLERQREITELKVKEFENIKLQLQENHEDEVKKVKAEVEDLKYLLDQSQKESQCLKSELQAQKEANSRAPTTTMRNLVERLKSQLALKEKQQKALSRALLELRAEMTAAAEERIISATSQKEAHLNVQQIVDRHTRELKTQVEDLNENLLKLKEALKTSKNRENSLTDNLNDLNNELQKKQKAYNKILREKEEIDQENDELKRQIKRLTSGLQGKPLTDNKQSLIEELQRKVKKLENQLEGKVEEVDLKPMKEKNAKEELIRWEEGKKWQAKIEGIRNKLKEKEGEVFTLTKQLNTLKDLFAKADKEKLTLQRKLKTTGMTVDQVLGIRALESEKELEELKKRNLDLENDILYMRAHQALPRDSVVEDLHLQNRYLQEKLHALEKQFSKDTYSKPSISGIESDDHCQREQELQKENLKLSSENIELKFQLEQANKDLPRLKNQVRDLKEMCEFLKKEKAEVQRKLGHVRGSGRSGKTIPELEKTIGLMKKVVEKVQRENEQLKKASGILTSEKMANIEQENEKLKAELEKLKAHLGHQLSMHYESKTKGTEKIIAENERLRKELKKETDAAEKLRIAKNNLEILNEKMTVQLEETGKRLQFAESRGPQLEGADSKSWKSIVVTRMYETKLKELETDIAKKNQSITDLKQLVKEATEREQKVNKYNEDLEQQIKILKHVPEGAETEQGLKRELQVLRLANHQLDKEKAELIHQIEANKDQSGAESTIPDADQLKEKIKDLETQLKMSDLEKQHLKEEIKKLKKELENFDPSFFEEIEDLKYNYKEEVKKNILLEEKVKKLSEQLGVELTSPVAASEEFEDEEESPVNFPIY

SEQ ID NO: 12 - DNA, 2973 bp, Homo sapiens
ttagtaaatggggaaattaacaggactttcttcttcatcttcaaactcttcagaagcagcaacagggctagttaattcaactcccaattgttctgaaagtttttttaccttctcttctaagagaatattcttcttcacttcttccttgtaattatacttaagatcttcaatttcttcaaaaaatgaaggatcaaaattttccagttcttttttcagcttctttatttcctccttcaaatgctgcttttctagatctgacattttgagctgtgtctctagatcttttattttttcctttagttgatcagcatcaggtatggtgctttcagctccactttggtccttgttagcttctatctgatggattaattctgctttctctttatccagctgatgattagctaatctaagaacttgaagctcccgtttaaggccttgctctgtctcagcaccttcaggaacatgtttaagaatcttaatctgttgttcaaggtcttcattgtatttgttaactttttgttctctctctgttgcttcttttacaagctgtttaaggtcagtaatgctttgattttttttggcaatatcagtttccaattcttttaacttggtttcatacattcttgtaaccacaatggatttccagctcttactgtcagcaccttcaagctgtggacctctgctttctgcaaactgcaatctcttaccagtctcttctagttgaactgtcatcttctcatttaatatctctaaattattctttgctatccgtaatttctctgcagcatcagtttcttttttaagttctttacgaagcctttcattttcagcaataattttttctgtgcctttggtcttggattcatagtgcatgctcaactgatgcccaagatgagctttaagtttttctaattcagccttcaatttttcattttcctgctcaatattagccattttttcactagtcaatattcctgatgcttttttcaactgttcattttctctctggactttttcaactacttttttcattaaaccaatggttttttccagttctgggattgtctttccacttctaccagaccctctaacatggccaagtttccgctgaacttctgctttttctttcttaagaaattcacacatttccttcaaatctctgacttgattctttaatcttggcaaatctttatttgcttgttcaagctgaaatttcagttcaatattttcagatgacaacttcaagttttccttctgaagctcctgttctctctgacaatgatcatctgactctattcctgaaattgaaggcttagaatatgtatcctttgaaaactgtttttctaaagcatgaagtttttcttggaggtatctattttgtaaatgtaaatcttctacaacagaatctcgaggaagagcttggtgggccctcatatacaatatatcattttctaagtcaagatttctcttttttaattcttccaattctttttctgactccaaagctcgtattcccaaaacctgatcaacagtcatgccagttgtttttagtttcctctgcaaagtaagtttctctttatcggctttggcaaaaagatccttcaaagtattcaactgctttgttaaagtaaagacttccccctctttctcttttaacttgtttcgaattccttctattttggcttgccactttttaccttcttcccacctaattaattcttctttagcattcttttctttcataggttttaggtctacttcctccacctttccctctaattggttctctagttttttaactttcctttggagttcttcaattagactttgtttattatctgtcaggggtttgccctgtaatccactggttagtcttttaatttgccttttcagttcatcattctcttgatcaatttcctctttctctctaagtattttattataggctttttgtttcttttgcagttcattatttaagtcattcaaattatcagttagtgagttttctctgtttttacttgttttaagtgcttctttcaattttaaaagattttcatttaaatcttcaacttgtgtctttagctctctagtatgtcgatcaacgatttgttgaacattgagatgggcctctttttgagaagttgcagaaataatacgttcttcagcagctgctgtcatttctgcccggagttctaaaagtgcccgactaagtgctttctgttgtttctccttcaaggctaattggctctttagccgttctactagatttctcattgtagttgttggagctcttgaatttgcttctttttgagcctgaagttcagattttaaacactgtgactccttttgtgactggtccagaagatactttaaatcctctacttccgcttttacttttttcacttcatcttcatggttttcttgaagctgtaatttgatattttcaaattcttttacttttaattcagtgatttctctttgtctctccaaatcttgtgatactttctttagtttgaccaagagtgaggaaagagagtcatcttgttctgctactgtctgttccatctcagccagacgaataaaatgcttgttggtaggaactggagtgggagactgtttcattaaatcccaagccgtttgtttgaatttatttagtgaactatcagcctgtagttctaatctgtgatgaagaatatgaaggtcttcctcatgtttcttcacaatttctctttgctcctctctggctttttctagaagacgttgatacttctttaatacttcttctttttgatttaaccttgcttgcatgtttgcaatggtttgatgagcaattttcaatgtgtggtgagattttggttccatctcttttctgcctagctcagctatgagcttttctctttctgcagtggcaggcaatcgaagcctcagttcattgattactttgtctcttgacagtatattttgttctgctaa

SEQ ID NO: 13 - DNA, 130 bp, adeno-associated virus 2
ctgcgcgctcgctcgctcactgaggccgcccgggcaaagcccgggcgtcgggcgacctttggtcgcccggcctcagtgagcgagcgagcgcgcagagagggagtggccaactccatcactaggggttcct

SEQ ID NO: 14 - DNA, 130 bp, adeno-associated virus 2
aggaacccctagtgatggagttggccactccctctctgcgcgctcgctcgctcactgaggccgggcgaccaaaggtcgcccgacgcccgggctttgcccgggcggcctcagtgagcgagcgagcgcgcag

SEQ ID NO: 15 - DNA, 6 bp, adeno-associated virus 2
agttgg

SEQ ID NO: 16 - DNA, 16 bp, adeno-associated virus 2
gcgcgctcgctcgctc

SEQ ID NO: 17 - DNA, 294 bp, Homo sapiens
gggccccagaagcctggtggttgtttgtccttctcaggggaaaagtgaggcggccccttggaggaaggggccgggcagaatgatctaatcggattccaagcagctcaggggattgtctttttctagcaccttcttgccactcctaagcgtcctccgtgaccccggctgggatttagcctggtgctgtgtcagccccgggctcccaggggcttcccagtggtccccaggaaccctcgacagggccagggcgtctctctcgtccagcaagggcagggacgggccacaggccaaggg

SEQ ID NO: 18 - DNA, 660 bp, Cytomegalovirus
cgcgtggagctagttattaatagtaatcaattacggggtcattagttcatagcccatatatggagttccgcgttacataacttacggtaaatggcccgcctggctgaccgcccaacgacccccgcccattgacgtcaataatgacgtatgttcccatagtaacgtcaatagggactttccattgacgtcaatgggtggagtatttacggtaaactgcccacttggcagtacatcaagtgtatcatatgccaagtacgccccctattgacgtcaatgacggtaaatggcccgcctggcattatgcccagtacatgaccttatgggactttcctacttggcagtacatctacgtattagtcatcgctattaccatggtgatgcggttttggcagtacatcaatgggcgtggatagcggtttgactcacggggatttccaagtctccaccccattgacgtcaatgggagtttgttttgcaccaaaatcaacgggactttccaaaatgtcgtaacaactccgccccattgacgcaaatgggcggtaggcgtgtacggtgggaggtctatataagcagagctcgtttagtgaaccgtcagatcgcctggagacgccatccacgctgttttgacctccatagaagacaccgggaccgatccagcct

SEQ ID NO: 19 - DNA, 2217 bp, Adeno-associated virus type 8
atggctgccgatggttatcttccagattggctcgaggacaacctctctgagggcattcgcgagtggtgggcgctgaaacctggagccccgaagcccaaagccaaccagcaaaagcaggacgacggccggggtctggtgcttcctggctacaagtacctcggacccttcaacggactcgacaagggggagcccgtcaacgcggcggacgcagcggccctcgagcacgacaaggcctacgaccagcagctgcaggcgggtgacaatccgtacctgcggtataaccacgccgacgccgagtttcaggagcgtctgcaagaagatacgtcttttgggggcaacctcgggcgagcagtcttccaggccaagaagcgggttctcgaacctctcggtctggttgaggaaggcgctaagacggctcctggaaagaagagaccggtagagccatcaccccagcgttctccagactcctctacgggcatcggcaagaaaggccaacagcccgccagaaaaagactcaattttggtcagactggcgactcagagtcagttccagaccctcaacctctcggagaacctccagcagcgccctctggtgtgggacctaatacaatggctgcaggcggtggcgcaccaatggcagacaataacgaaggcgccgacggagtgggtagttcctcgggaaattggcattgcgattccacatggctgggcgacagagtcatcaccaccagcacccgaacctgggccctgcccacctacaacaaccacctctacaagcaaatctccaacgggacatcgggaggagccaccaacgacaacacctacttcggctacagcaccccctgggggtattttgactttaacagattccactgccacttttcaccacgtgactggcagcgactcatcaacaacaactggggattccggcccaagagactcagcttcaagctcttcaacatccaggtcaaggaggtcacgcagaatgaaggcaccaagaccatcgccaataacctcaccagcaccatccaggtgtttacggactcggagtaccagctgccgtacgttctcggctctgcccaccagggctgcctgcctccgttcccggcggacgtgttcatgattccccagtacggctacctaacactcaacaacggtagtcaggccgtgggacgctcctccttctactgcctggaatactttccttcgcagatgctgagaaccggcaacaacttccagtttacttacaccttcgaggacgtgcctttccacagcagctacgcccacagccagagcttggaccggctgatgaatcctctgattgaccagtacctgtactacttgtctcggactcaaacaacaggaggcacggcaaatacgcagactctgggcttcagccaaggtgggcctaatacaatggccaatcaggcaaagaactggctgccaggaccctgttaccgccaacaacgcgtctcaacgacaaccgggcaaaacaacaatagcaactttgcctggactgctgggaccaaataccatctgaatggaagaaattcattggctaatcctggcatcgctatggcaacacacaaagacgacgaggagcgtttttttcccagtaacgggatcctgatttttggcaaacaaaatgctgccagagacaatgcggattacagcgatgtcatgctcaccagcgaggaagaaatcaaaaccactaaccctgtggctacagaggaatacggtatcgtggcagataacttgcagcagcaaaacacggctcctcaaattggaactgtcaacagccagggggccttacccggtatggtctggcagaaccgggacgtgtacctgcagggtcccatctgggccaagattcctcacacggacggcaacttccacccgtctccgctgatgggcggctttggcctgaaacatcctccgcctcagatcctgatcaagaacacgcctgtacctgcggatcctccgaccaccttcaaccagtcaaagctgaactctttcatcacgcaatacagcaccggacaggtcagcgtggaaattgaatgggagctgcagaaggaaaacagcaagcgctggaaccccgagatccagtacacctccaactactacaaatctacaagtgtggactttgctgttaatacagaaggcgtgtactctgaaccccgccccattggcacccgttacctcacccgtaatctgtaa

SEQ ID NO: 20 - protein, 738 aa, Adeno-associated virus type 8
MAADGYLPDWLEDNLSEGIREWWALKPGAPKPKANQQKQDDGRGLVLPGYKYLGPFNGLDKGEPVNAADAAALEHDKAYDQQLQAGDNPYLRYNHADAEFQERLQEDTSFGGNLGRAVFQAKKRVLEPLGLVEEGAKTAPGKKRPVEPSPQRSPDSSTGIGKKGQQPARKRLNFGQTGDSESVPDPQPLGEPPAAPSGVGPNTMAAGGGAPMADNNEGADGVGSSSGNWHCDSTWLGDRVITTSTRTWALPTYNNHLYKQISNGTSGGATNDNTYFGYSTPWGYFDFNRFHCHFSPRDWQRLINNNWGFRPKRLSFKLFNIQVKEVTQNEGTKTIANNLTSTIQVFTDSEYQLPYVLGSAHQGCLPPFPADVFMIPQYGYLTLNNGSQAVGRSSFYCLEYFPSQMLRTGNNFQFTYTFEDVPFHSSYAHSQSLDRLMNPLIDQYLYYLSRTQTTGGTANTQTLGFSQGGPNTMANQAKNWLPGPCYRQQRVSTTTGQNNNSNFAWTAGTKYHLNGRNSLANPGIAMATHKDDEERFFPSNGILIFGKQNAARDNADYSDVMLTSEEEIKTTNPVATEEYGIVADNLQQQNTAPQIGTVNSQGALPGMVWQNRDVYLQGPIWAKIPHTDGNFHPSPLMGGFGLKHPPPQILIKNTPVPADPPTTFNQSKLNSFITQYSTGQVSVEIEWELQKENSKRWNPEIQYTSNYYKSTSVDFAVNTEGVYSEPRPIGTRYLTRNL

SEQ ID NO: 21 - DNA, 294 bp, Adeno-associated virus type 8
cccttggcctgtggcccgtccctgcccttgctggacgagagagacgccctggccctgtcgagggttcctggggaccactgggaagcccctgggagcccggggctgacacagcaccaggctaaatcccagccggggtcacggaggacgcttaggagtggcaagaaggtgctagaaaaagacaatcccctgagctgcttggaatccgattagatcattctgcccggccccttcctccaaggggccgcctcacttttcccctgagaaggacaaacaaccaccaggcttctggggccc

SEQ ID NO: 22 - DNA, 897 bp, Mus musculus
gatttacttaagcagtctcctgctccagttcccaccaacaaacatttcattcgtctggccgagatggagcagacagtagcagaacaagatgactctctgtcctcacttttgaccaaactaaagaaagtatcaaaagatttggaaaaacaaaaagaaatcactgagttaaaagtcagagagtttgaaaataccaaactacggctccaagaaactcatgccagtgaggtaaagaaagtgaaagcagaggtagaggacttaaggcatgctctagcccaagcacacaaggactcccagagtttaaagtctgaactccaggctcagaaagaagcaaactccagagctccaacaaccacaatgaggaatcttgtagacaggctaaagagccaactagccttgaaagagaagcaacaaaaggcacttagtcgagccctgttggaacttcggtcggaaatgacagcagcagctgaggaacgtataatcgctgtaacttctcaaaaagaggcaaatctcaatgttcaacaagttgttgagcgccatactagagagctaaagtcacaaattgaagatttaaatgaaaatcttttaaaattgaaagaagctcttaaaacaagtaagaacaaagaaaattcactagctgatgatttaaatgaattaaataatgaactgcaaaaaaagcaaaaagcttataataaaatccttagagagaaagatggaattgatcaagaaaatgatgaactgagaagacagattaaaagactgtccagtggactgcagagcaaaactttgatagataacaagcaaagtttaatcgatgaacttcaaaagaaagttaaaaaacttgaaagccaactggaaagaaaggtggatgacgtagacataaagccggtgaaggaaaag

SEQ ID NO: 23 - protein, 299 aa, Mus musculus
DLLKQSPAPVPTNKHFIRLAEMEQTVAEQDDSLSSLLTKLKKVSKDLEKQKEITELKVREFENTKLRLQETHASEVKKVKAEVEDLRHALAQAHKDSQSLKSELQAQKEANSRAPTTTMRNLVDRLKSQLALKEKQQKALSRALLELRSEMTAAAEERIIAVTSQKEANLNVQQVVERHTRELKSQIEDLNENLLKLKEALKTSKNKENSLADDLNELNNELQKKQKAYNKILREKDGIDQENDELRRQIKRLSSGLQSKTLIDNKQSLIDELQKKVKKLESQLERKVDDVDIKPVKEK

SEQ ID NO: 24 - DNA, 897 bp, Mus musculus
cttttccttcaccggctttatgtctacgtcatccacctttctttccagttggctttcaagttttttaactttcttttgaagttcatcgattaaactttgcttgttatctatcaaagttttgctctgcagtccactggacagtcttttaatctgtcttctcagttcatcattttcttgatcaattccatctttctctctaaggattttattataagctttttgctttttttgcagttcattatttaattcatttaaatcatcagctagtgaattttctttgttcttacttgttttaagagcttctttcaattttaaaagattttcatttaaatcttcaatttgtgactttagctctctagtatggcgctcaacaacttgttgaacattgagatttgcctctttttgagaagttacagcgattatacgttcctcagctgctgctgtcatttccgaccgaagttccaacagggctcgactaagtgccttttgttgcttctctttcaaggctagttggctctttagcctgtctacaagattcctcattgtggttgttggagctctggagtttgcttctttctgagcctggagttcagactttaaactctgggagtccttgtgtgcttgggctagagcatgccttaagtcctctacctctgctttcactttctttacctcactggcatgagtttcttggagccgtagtttggtattttcaaactctctgacttttaactcagtgatttctttttgtttttccaaatcttttgatactttctttagtttggtcaaaagtgaggacagagagtcatcttgttctgctactgtctgctccatctcggccagacgaatgaaatgtttgttggtgggaactggagcaggagactgcttaagtaaatc

SEQ ID NO: 25 - DNA, 897 bp, Homo sapiens
gatttaatgaaacagtctcccactccagttcctaccaacaagcattttattcgtctggctgagatggaacagacagtagcagaacaagatgactctctttcctcactcttggtcaaactaaagaaagtatcacaagatttggagagacaaagagaaatcactgaattaaaagtaaaagaatttgaaaatatcaaattacagcttcaagaaaaccatgaagatgaagtgaaaaaagtaaaagcggaagtagaggatttaaagtatcttctggaccagtcacaaaaggagtcacagtgtttaaaatctgaacttcaggctcaaaaagaagcaaattcaagagctccaacaactacaatgagaaatctagtagaacggctaaagagccaattagccttgaaggagaaacaacagaaagcacttagtcgggcacttttagaactccgggcagaaatgacagcagctgctgaagaacgtattatttctgcaacttctcaaaaagaggcccatctcaatgttcaacaaatcgttgatcgacatactagagagctaaagacacaagttgaagatttaaatgaaaatcttttaaaattgaaagaagcacttaaaacaagtaaaaacagagaaaactcactaactgataatttgaatgacttaaataatgaactgcaaaagaaacaaaaagcctataataaaatacttagagagaaagaggaaattgatcaagagaatgatgaactgaaaaggcaaattaaaagactaaccagtggattacagggcaaacccctgacagataataaacaaagtctaattgaagaactccaaaggaaagttaaaaaactagagaaccaattagagggaaaggtggaggaagtagacctaaaacctatgaaagaaaag

SEQ ID NO: 26 - protein, 299 aa, Homo sapiens
DLMKQSPTPVPTNKHFIRLAEMEQTVAEQDDSLSSLLVKLKKVSQDLERQREITELKVKEFENIKLQLQENHEDEVKKVKAEVEDLKYLLDQSQKESQCLKSELQAQKEANSRAPTTTMRNLVERLKSQLALKEKQQKALSRALLELRAEMTAAAEERIISATSQKEAHLNVQQIVDRHTRELKTQVEDLNENLLKLKEALKTSKNRENSLTDNLNDLNNELQKKQKAYNKILREKEEIDQENDELKRQIKRLTSGLQGKPLTDNKQSLIEELQRKVKKLENQLEGKVEEVDLKPMKEK

SEQ ID NO: 27 - DNA, 897 bp, Homo sapiens
cttttctttcataggttttaggtctacttcctccacctttccctctaattggttctctagttttttaactttcctttggagttcttcaattagactttgtttattatctgtcaggggtttgccctgtaatccactggttagtcttttaatttgccttttcagttcatcattctcttgatcaatttcctctttctctctaagtattttattataggctttttgtttcttttgcagttcattatttaagtcattcaaattatcagttagtgagttttctctgtttttacttgttttaagtgcttctttcaattttaaaagattttcatttaaatcttcaacttgtgtctttagctctctagtatgtcgatcaacgatttgttgaacattgagatgggcctctttttgagaagttgcagaaataatacgttcttcagcagctgctgtcatttctgcccggagttctaaaagtgcccgactaagtgctttctgttgtttctccttcaaggctaattggctctttagccgttctactagatttctcattgtagttgttggagctcttgaatttgcttctttttgagcctgaagttcagattttaaacactgtgactccttttgtgactggtccagaagatactttaaatcctctacttccgcttttacttttttcacttcatcttcatggttttcttgaagctgtaatttgatattttcaaattcttttacttttaattcagtgatttctctttgtctctccaaatcttgtgatactttctttagtttgaccaagagtgaggaaagagagtcatcttgttctgctactgtctgttccatctcagccagacgaataaaatgcttgttggtaggaactggagtgggagactgtttcattaaatc

SEQ ID NO: 28 - DNA, 3924 bp, Mus musculus
caacaacagtccagggaaaaggaagtggaatccctcagaacgcagctgctggacttccaggcacaatctgacgaaaaggctctaattgccaaattgcaccaacatgttgtctctcttcaaattagtgaggccactgccctcggtaagttagagtcagttacgtccaaactccagaagatggaagcctacaatttgcgcttagaacagaaactggatgaaaaagagcaggcgctctactatgctcgtttggaaggtagaaacagagcaaaacacctgcgccaaaccattcagtcgcttcgaagacagttcagtggagctctacccttagcacagcaggaaaagttctccaaaacgatgattcagttgcaaaatgacaaacttaagataatgcaagaaatgaagaattcgcaacaggaacacagaaatatggaaaacaaaacactggagttggaattaaaattaaaaggcttagaagaattgatcagtactttaaaggatgccaggggagcccagaaggtaatcaattggcatgtgaaaatagaagaacttcgcctccaagaacttaagctaaatagagaactagtcaagggtaaagaagaaatcaaatatttgaataatatcatctctgaatatgagcatacaatcaacagtctagaggaagaaattgttcagcaaagcaagttccatgaagaaagacagatggcttgggatcaaagagaagttgagctggaacgccagttagacatttttgatcatcagcaaaatgaaatactcagtgcagcacaaaagtttgaagactctacaggatcaatgccagaccccagcttgcctcttccaaaccaacttgaaattgctctaagaaaaattaaggagaatattcaagtaattcttaaaacacaagcaacttgcaagtcactagaagagaaactaaaagaaaaagaatctgctttacggttggcagagcaaaatattctgtcaagagacaaagtaatcaatgaactgaggcttcgattgcctgccacggctgatcgagaaaaacttatagctgagctagaaagaaaagagctggagccgaaatctcatcacacaatgaaaattgcccaccaaactattgccaacatgcaggcaaggttaaatcacaaggaagaagtattgaagaaataccagcaccttctggagaaggccagagaggagcaaagagaaattgttaagaagcatgaggaagaccttcatgttcttcatcacaaattagaacaacaggccgataattcactcaataaattcagacagacagctcaggatttacttaagcagtctcctgctccagttcccaccaacaaacatttcattcgtctggccgagatggagcagacagtagcagaacaagatgactctctgtcctcacttttgaccaaactaaagaaagtatcaaaagatttggaaaaacaaaaagaaatcactgagttaaaagtcagagagtttgaaaataccaaactacggctccaagaaactcatgccagtgaggtaaagaaagtgaaagcagaggtagaggacttaaggcatgctctagcccaagcacacaaggactcccagagtttaaagtctgaactccaggctcagaaagaagcaaactccagagctccaacaaccacaatgaggaatcttgtagacaggctaaagagccaactagccttgaaagagaagcaacaaaaggcacttagtcgagccctgttggaacttcggtcggaaatgacagcagcagctgaggaacgtataatcgctgtaacttctcaaaaagaggcaaatctcaatgttcaacaagttgttgagcgccatactagagagctaaagtcacaaattgaagatttaaatgaaaatcttttaaaattgaaagaagctcttaaaacaagtaagaacaaagaaaattcactagctgatgatttaaatgaattaaataatgaactgcaaaaaaagcaaaaagcttataataaaatccttagagagaaagatggaattgatcaagaaaatgatgaactgagaagacagattaaaagactgtccagtggactgcagagcaaaactttgatagataacaagcaaagtttaatcgatgaacttcaaaagaaagttaaaaaacttgaaagccaactggaaagaaaggtggatgacgtagacataaagccggtgaaggaaaagagtagtaaagaagaattaattaggtgggaagaaggtaagaaatggcaaaccaaagtagagggactacgaaacagactaaaggagaaggaaggagaagcccacggcctggcaaagcagctgaataccttaaaggaactttttgccaaagctgataaagagaaacttactttgcagaagaaactgaaaacaacaggaatgactgttgaccaggttttaggagtgcgagctttggaatctgaaaaagagttggaagagctaaaaaagaaaaatctggacctagaaaatgacatattatacatgaggacccagcaggctcttccacgagattctgttgtggaagacttacatttacaaaataaataccttcaagaaaaacttcatactttagaaaaaaaactttcaaaggagaaatattctcagtctttgacttcagaaatagagtcagatgatcactgtcaaaaagaacaagaacttcagaaggaaaatttgaagttgtcatctgaaaacatcgagctgaaatttcaacttgaacaagcaaataaagatttgccaagactaaagaatcaagtgaaagatttgaaggaaatgtgtgaatttcttaagaaaggaaaactggaacttgagcggaagcttggtcaggtcagaggggctggtagaagtgggaagacaatcccagaactagaaaaaaccattgggttaatgaagaaagtagttgaaaaagtccaaagagaaaatgaacaattgaaaaaggcatcaggaatactgactagtgaaaaaatggctactattgaggaagaaaatagaaacttaaaggctgaactagaaaagcttaaagctcactttggacgtcagttgagtatgcagtttgaatctaagaacaaaggtactgagaaaattgttgccgaaaatgaacggcttcggaaagaacttaagaaagaaatagaagcctctgagaaactgcggatagctaagaacaacttagagctggtgaacgacaagatggcagctcaactcgaagaaactgggaagagactacagtttgcagaaagtagagccccacagctggaaggtgctgacagcaagagctggaagtcaattgtggtctcaagagtgtatgagaccaagatgaaagagcttgaaagtgacattgccaaaaagaatcaaagtatcactgaccttaaacagcttgtaagagaagcaacagagagagaacagaaagctaagaaatacactgaagaccttgaacaacagattgagatcctcaaaaatgttcctgaaggtgccgagacagagcaagagcttatacgggaactccagcttcttagattagccaataatcagatggataaagaaagggcagaattaatccatcagatagaaattaacaaggaccaaaccagagctgacagtagcatacctgattctgatcaactaaaggaaaagataaatgacctggagacacaactcagaaagttggagctagaaaagcaacattcgaaggaggaagttaaaaagctgaaaaaagaactggaaaattttgatccttcattttttgaagaaattgaagacctgaagtataattataaggaagaagtgaaaaagaatatcctattagaagagaagctaaaaaaactgtcggaacagtttggatttgaactgcctagtcctcttgctgcttctgaacactcggaagatggagaaagtcctcatagtttccctatttattag

SEQ ID NO: 29 - protein, 1307 aa, Mus musculus
QQQSREKEVESLRTQLLDFQAQSDEKALIAKLHQHVVSLQISEATALGKLESVTSKLQKMEAYNLRLEQKLDEKEQALYYARLEGRNRAKHLRQTIQSLRRQFSGALPLAQQEKFSKTMIQLQNDKLKIMQEMKNSQQEHRNMENKTLELELKLKGLEELISTLKDARGAQKVINWHVKIEELRLQELKLNRELVKGKEEIKYLNNIISEYEHTINSLEEEIVQQSKFHEERQMAWDQREVELERQLDIFDHQQNEILSAAQKFEDSTGSMPDPSLPLPNQLEIALRKIKENIQVILKTQATCKSLEEKLKEKESALRLAEQNILSRDKVINELRLRLPATADREKLIAELERKELEPKSHHTMKIAHQTIANMQARLNHKEEVLKKYQHLLEKAREEQREIVKKHEEDLHVLHHKLEQQADNSLNKFRQTAQDLLKQSPAPVPTNKHFIRLAEMEQTVAEQDDSLSSLLTKLKKVSKDLEKQKEITELKVREFENTKLRLQETHASEVKKVKAEVEDLRHALAQAHKDSQSLKSELQAQKEANSRAPTTTMRNLVDRLKSQLALKEKQQKALSRALLELRSEMTAAAEERIIAVTSQKEANLNVQQVVERHTRELKSQIEDLNENLLKLKEALKTSKNKENSLADDLNELNNELQKKQKAYNKILREKDGIDQENDELRRQIKRLSSGLQSKTLIDNKQSLIDELQKKVKKLESQLERKVDDVDIKPVKEKSSKEELIRWEEGKKWQTKVEGLRNRLKEKEGEAHGLAKQLNTLKELFAKADKEKLTLQKKLKTTGMTVDQVLGVRALESEKELEELKKKNLDLENDILYMRTQQALPRDSVVEDLHLQNKYLQEKLHTLEKKLSKEKYSQSLTSEIESDDHCQKEQELQKENLKLSSENIELKFQLEQANKDLPRLKNQVKDLKEMCEFLKKGKLELERKLGQVRGAGRSGKTIPELEKTIGLMKKVVEKVQRENEQLKKASGILTSEKMATIEEENRNLKAELEKLKAHFGRQLSMQFESKNKGTEKIVAENERLRKELKKEIEASEKLRIAKNNLELVNDKMAAQLEETGKRLQFAESRAPQLEGADSKSWKSIVVSRVYETKMKELESDIAKKNQSITDLKQLVREATEREQKAKKYTEDLEQQIEILKNVPEGAETEQELIRELQLLRLANNQMDKERAELIHQIEINKDQTRADSSIPDSDQLKEKINDLETQLRKLELEKQHSKEEVKKLKKELENFDPSFFEEIEDLKYNYKEEVKKNILLEEKLKKLSEQFGFELPSPLAASEHSEDGESPHSFPIY

SEQ ID NO: 30 - DNA, 3924 bp, Mus musculus
ctaataaatagggaaactatgaggactttctccatcttccgagtgttcagaagcagcaagaggactaggcagttcaaatccaaactgttccgacagtttttttagcttctcttctaataggatattctttttcacttcttccttataattatacttcaggtcttcaatttcttcaaaaaatgaaggatcaaaattttccagttcttttttcagctttttaacttcctccttcgaatgttgcttttctagctccaactttctgagttgtgtctccaggtcatttatcttttcctttagttgatcagaatcaggtatgctactgtcagctctggtttggtccttgttaatttctatctgatggattaattctgccctttctttatccatctgattattggctaatctaagaagctggagttcccgtataagctcttgctctgtctcggcaccttcaggaacatttttgaggatctcaatctgttgttcaaggtcttcagtgtatttcttagctttctgttctctctctgttgcttctcttacaagctgtttaaggtcagtgatactttgattctttttggcaatgtcactttcaagctctttcatcttggtctcatacactcttgagaccacaattgacttccagctcttgctgtcagcaccttccagctgtggggctctactttctgcaaactgtagtctcttcccagtttcttcgagttgagctgccatcttgtcgttcaccagctctaagttgttcttagctatccgcagtttctcagaggcttctatttctttcttaagttctttccgaagccgttcattttcggcaacaattttctcagtacctttgttcttagattcaaactgcatactcaactgacgtccaaagtgagctttaagcttttctagttcagcctttaagtttctattttcttcctcaatagtagccattttttcactagtcagtattcctgatgcctttttcaattgttcattttctctttggactttttcaactactttcttcattaacccaatggttttttctagttctgggattgtcttcccacttctaccagcccctctgacctgaccaagcttccgctcaagttccagttttcctttcttaagaaattcacacatttccttcaaatctttcacttgattctttagtcttggcaaatctttatttgcttgttcaagttgaaatttcagctcgatgttttcagatgacaacttcaaattttccttctgaagttcttgttctttttgacagtgatcatctgactctatttctgaagtcaaagactgagaatatttctcctttgaaagttttttttctaaagtatgaagtttttcttgaaggtatttattttgtaaatgtaagtcttccacaacagaatctcgtggaagagcctgctgggtcctcatgtataatatgtcattttctaggtccagatttttcttttttagctcttccaactctttttcagattccaaagctcgcactcctaaaacctggtcaacagtcattcctgttgttttcagtttcttctgcaaagtaagtttctctttatcagctttggcaaaaagttcctttaaggtattcagctgctttgccaggccgtgggcttctccttccttctcctttagtctgtttcgtagtccctctactttggtttgccatttcttaccttcttcccacctaattaattcttctttactactcttttccttcaccggctttatgtctacgtcatccacctttctttccagttggctttcaagttttttaactttcttttgaagttcatcgattaaactttgcttgttatctatcaaagttttgctctgcagtccactggacagtcttttaatctgtcttctcagttcatcattttcttgatcaattccatctttctctctaaggattttattataagctttttgctttttttgcagttcattatttaattcatttaaatcatcagctagtgaattttctttgttcttacttgttttaagagcttctttcaattttaaaagattttcatttaaatcttcaatttgtgactttagctctctagtatggcgctcaacaacttgttgaacattgagatttgcctctttttgagaagttacagcgattatacgttcctcagctgctgctgtcatttccgaccgaagttccaacagggctcgactaagtgccttttgttgcttctctttcaaggctagttggctctttagcctgtctacaagattcctcattgtggttgttggagctctggagtttgcttctttctgagcctggagttcagactttaaactctgggagtccttgtgtgcttgggctagagcatgccttaagtcctctacctctgctttcactttctttacctcactggcatgagtttcttggagccgtagtttggtattttcaaactctctgacttttaactcagtgatttctttttgtttttccaaatcttttgatactttctttagtttggtcaaaagtgaggacagagagtcatcttgttctgctactgtctgctccatctcggccagacgaatgaaatgtttgttggtgggaactggagcaggagactgcttaagtaaatcctgagctgtctgtctgaatttattgagtgaattatcggcctgttgttctaatttgtgatgaagaacatgaaggtcttcctcatgcttcttaacaatttctctttgctcctctctggccttctccagaaggtgctggtatttcttcaatacttcttccttgtgatttaaccttgcctgcatgttggcaatagtttggtgggcaattttcattgtgtgatgagatttcggctccagctcttttctttctagctcagctataagtttttctcgatcagccgtggcaggcaatcgaagcctcagttcattgattactttgtctcttgacagaatattttgctctgccaaccgtaaagcagattctttttcttttagtttctcttctagtgacttgcaagttgcttgtgttttaagaattacttgaatattctccttaatttttcttagagcaatttcaagttggtttggaagaggcaagctggggtctggcattgatcctgtagagtcttcaaacttttgtgctgcactgagtatttcattttgctgatgatcaaaaatgtctaactggcgttccagctcaacttctctttgatcccaagccatctgtctttcttcatggaacttgctttgctgaacaatttcttcctctagactgttgattgtatgctcatattcagagatgatattattcaaatatttgatttcttctttacccttgactagttctctatttagcttaagttcttggaggcgaagttcttctattttcacatgccaattgattaccttctgggctcccctggcatcctttaaagtactgatcaattcttctaagccttttaattttaattccaactccagtgttttgttttccatatttctgtgttcctgttgcgaattcttcatttcttgcattatcttaagtttgtcattttgcaactgaatcatcgttttggagaacttttcctgctgtgctaagggtagagctccactgaactgtcttcgaagcgactgaatggtttggcgcaggtgttttgctctgtttctaccttccaaacgagcatagtagagcgcctgctctttttcatccagtttctgttctaagcgcaaattgtaggcttccatcttctggagtttggacgtaactgactctaacttaccgagggcagtggcctcactaatttgaagagagacaacatgttggtgcaatttggcaattagagccttttcgtcagattgtgcctggaagtccagcagctgcgttctgagggattccacttccttttccctggactgttgttg

SEQ ID NO: 31 - DNA, 3924 bp, Homo sapiens
caacaatctagggacaaggaagtagagtccctcagaatgcaactgctagactatcaggcacagtctgatgaaaagtcgctcattgccaagttgcaccaacataatgtctctcttcaactgagtgaggctactgctcttggtaagttggagtcaattacatctaaactgcagaagatggaggcctacaacttgcgcttagagcagaaacttgatgaaaaagaacaggctctctattatgctcgtttggagggaagaaacagagcaaaacatctgcgccaaacaattcagtctctacgacgacagtttagtggagctttacccttggcacaacaggaaaagttctccaaaacaatgattcaactacaaaatgacaaacttaagataatgcaagaaatgaaaaattctcaacaagaacatagaaatatggagaacaaaacattggagatggaattaaaattaaagggcctggaagagttaataagcactttaaaggataccaaaggagcccaaaaggtaatcaactggcatatgaaaatagaagaacttcgtcttcaagaacttaaactaaatcgggaattagtcaaggataaagaagaaataaaatatttgaataacataatttctgaatatgaacgtacaatcagcagtcttgaagaagaaattgtgcaacagaacaagtttcatgaagaaagacaaatggcctgggatcaaagagaagttgacctggaacgccaactagacatttttgaccgtcagcaaaatgaaatactaaatgcggcacaaaagtttgaagaagctacaggatcaatccctgaccctagtttgccccttccaaatcaacttgagatcgctctaaggaaaattaaggagaacattcgaataattctagaaacacgggcaacttgcaaatcactagaagagaaactaaaagagaaagaatctgctttaaggttagcagaacaaaatatactgtcaagagacaaagtaatcaatgaactgaggcttcgattgcctgccactgcagaaagagaaaagctcatagctgagctaggcagaaaagagatggaaccaaaatctcaccacacattgaaaattgctcatcaaaccattgcaaacatgcaagcaaggttaaatcaaaaagaagaagtattaaagaagtatcaacgtcttctagaaaaagccagagaggagcaaagagaaattgtgaagaaacatgaggaagaccttcatattcttcatcacagattagaactacaggctgatagttcactaaataaattcaaacaaacggcttgggatttaatgaaacagtctcccactccagttcctaccaacaagcattttattcgtctggctgagatggaacagacagtagcagaacaagatgactctctttcctcactcttggtcaaactaaagaaagtatcacaagatttggagagacaaagagaaatcactgaattaaaagtaaaagaatttgaaaatatcaaattacagcttcaagaaaaccatgaagatgaagtgaaaaaagtaaaagcggaagtagaggatttaaagtatcttctggaccagtcacaaaaggagtcacagtgtttaaaatctgaacttcaggctcaaaaagaagcaaattcaagagctccaacaactacaatgagaaatctagtagaacggctaaagagccaattagccttgaaggagaaacaacagaaagcacttagtcgggcacttttagaactccgggcagaaatgacagcagctgctgaagaacgtattatttctgcaacttctcaaaaagaggcccatctcaatgttcaacaaatcgttgatcgacatactagagagctaaagacacaagttgaagatttaaatgaaaatcttttaaaattgaaagaagcacttaaaacaagtaaaaacagagaaaactcactaactgataatttgaatgacttaaataatgaactgcaaaagaaacaaaaagcctataataaaatacttagagagaaagaggaaattgatcaagagaatgatgaactgaaaaggcaaattaaaagactaaccagtggattacagggcaaacccctgacagataataaacaaagtctaattgaagaactccaaaggaaagttaaaaaactagagaaccaattagagggaaaggtggaggaagtagacctaaaacctatgaaagaaaagaatgctaaagaagaattaattaggtgggaagaaggtaaaaagtggcaagccaaaatagaaggaattcgaaacaagttaaaagagaaagagggggaagtctttactttaacaaagcagttgaatactttgaaggatctttttgccaaagccgataaagagaaacttactttgcagaggaaactaaaaacaactggcatgactgttgatcaggttttgggaatacgagctttggagtcagaaaaagaattggaagaattaaaaaagagaaatcttgacttagaaaatgatatattgtatatgagggcccaccaagctcttcctcgagattctgttgtagaagatttacatttacaaaatagatacctccaagaaaaacttcatgctttagaaaaacagttttcaaaggatacatattctaagccttcaatttcaggaatagagtcagatgatcattgtcagagagaacaggagcttcagaaggaaaacttgaagttgtcatctgaaaatattgaactgaaatttcagcttgaacaagcaaataaagatttgccaagattaaagaatcaagtcagagatttgaaggaaatgtgtgaatttcttaagaaagaaaaagcagaagttcagcggaaacttggccatgttagagggtctggtagaagtggaaagacaatcccagaactggaaaaaaccattggtttaatgaaaaaagtagttgaaaaagtccagagagaaaatgaacagttgaaaaaagcatcaggaatattgactagtgaaaaaatggctaatattgagcaggaaaatgaaaaattgaaggctgaattagaaaaacttaaagctcatcttgggcatcagttgagcatgcactatgaatccaagaccaaaggcacagaaaaaattattgctgaaaatgaaaggcttcgtaaagaacttaaaaaagaaactgatgctgcagagaaattacggatagcaaagaataatttagagatattaaatgagaagatgacagttcaactagaagagactggtaagagattgcagtttgcagaaagcagaggtccacagcttgaaggtgctgacagtaagagctggaaatccattgtggttacaagaatgtatgaaaccaagttaaaagaattggaaactgatattgccaaaaaaaatcaaagcattactgaccttaaacagcttgtaaaagaagcaacagagagagaacaaaaagttaacaaatacaatgaagaccttgaacaacagattaagattcttaaacatgttcctgaaggtgctgagacagagcaaggccttaaacgggagcttcaagttcttagattagctaatcatcagctggataaagagaaagcagaattaatccatcagatagaagctaacaaggaccaaagtggagctgaaagcaccatacctgatgctgatcaactaaaggaaaaaataaaagatctagagacacagctcaaaatgtcagatctagaaaagcagcatttgaaggaggaaataaagaagctgaaaaaagaactggaaaattttgatccttcattttttgaagaaattgaagatcttaagtataattacaaggaagaagtgaagaagaatattctcttagaagagaaggtaaaaaaactttcagaacaattgggagttgaattaactagccctgttgctgcttctgaagagtttgaagatgaagaagaaagtcctgttaatttccccatttactaa

SEQ ID NO: 32 - protein, 1307 aa, Homo sapiens
QQSRDKEVESLRMQLLDYQAQSDEKSLIAKLHQHNVSLQLSEATALGKLESITSKLQKMEAYNLRLEQKLDEKEQALYYARLEGRNRAKHLRQTIQSLRRQFSGALPLAQQEKFSKTMIQLQNDKLKIMQEMKNSQQEHRNMENKTLEMELKLKGLEELISTLKDTKGAQKVINWHMKIEELRLQELKLNRELVKDKEEIKYLNNIISEYERTISSLEEEIVQQNKFHEERQMAWDQREVDLERQLDIFDRQQNEILNAAQKFEEATGSIPDPSLPLPNQLEIALRKIKENIRIILETRATCKSLEEKLKEKESALRLAEQNILSRDKVINELRLRLPATAEREKLIAELGRKEMEPKSHHTLKIAHQTIANMQARLNQKEEVLKKYQRLLEKAREEQREIVKKHEEDLHILHHRLELQADSSLNKFKQTAWDLMKQSPTPVPTNKHFIRLAEMEQTVAEQDDSLSSLLVKLKKVSQDLERQREITELKVKEFENIKLQLQENHEDEVKKVKAEVEDLKYLLDQSQKESQCLKSELQAQKEANSRAPTTTMRNLVERLKSQLALKEKQQKALSRALLELRAEMTAAAEERIISATSQKEAHLNVQQIVDRHTRELKTQVEDLNENLLKLKEALKTSKNRENSLTDNLNDLNNELQKKQKAYNKILREKEEIDQENDELKRQIKRLTSGLQGKPLTDNKQSLIEELQRKVKKLENQLEGKVEEVDLKPMKEKNAKEELIRWEEGKKWQAKIEGIRNKLKEKEGEVFTLTKQLNTLKDLFAKADKEKLTLQRKLKTTGMTVDQVLGIRALESEKELEELKKRNLDLENDILYMRAHQALPRDSVVEDLHLQNRYLQEKLHALEKQFSKDTYSKPSISGIESDDHCQREQELQKENLKLSSENIELKFQLEQANKDLPRLKNQVRDLKEMCEFLKKEKAEVQRKLGHVRGSGRSGKTIPELEKTIGLMKKVVEKVQRENEQLKKASGILTSEKMANIEQENEKLKAELEKLKAHLGHQLSMHYESKTKGTEKIIAENERLRKELKKETDAAEKLRIAKNNLEILNEKMTVQLEETGKRLQFAESRGPQLEGADSKSWKSIVVTRMYETKLKELETDIAKKNQSITDLKQLVKEATEREQKVNKYNEDLEQQIKILKHVPEGAETEQGLKRELQVLRLANHQLDKEKAELIHQIEANKDQSGAESTIPDADQLKEKIKDLETQLKMSDLEKQHLKEEIKKLKKELENFDPSFFEEIEDLKYNYKEEVKKNILLEEKVKKLSEQLGVELTSPVAASEEFEDEEESPVNFPIY

SEQ ID NO: 33 - DNA, 3924 bp, Homo sapiens
ttagtaaatggggaaattaacaggactttcttcttcatcttcaaactcttcagaagcagcaacagggctagttaattcaactcccaattgttctgaaagtttttttaccttctcttctaagagaatattcttcttcacttcttccttgtaattatacttaagatcttcaatttcttcaaaaaatgaaggatcaaaattttccagttcttttttcagcttctttatttcctccttcaaatgctgcttttctagatctgacattttgagctgtgtctctagatcttttattttttcctttagttgatcagcatcaggtatggtgctttcagctccactttggtccttgttagcttctatctgatggattaattctgctttctctttatccagctgatgattagctaatctaagaacttgaagctcccgtttaaggccttgctctgtctcagcaccttcaggaacatgtttaagaatcttaatctgttgttcaaggtcttcattgtatttgttaactttttgttctctctctgttgcttcttttacaagctgtttaaggtcagtaatgctttgattttttttggcaatatcagtttccaattcttttaacttggtttcatacattcttgtaaccacaatggatttccagctcttactgtcagcaccttcaagctgtggacctctgctttctgcaaactgcaatctcttaccagtctcttctagttgaactgtcatcttctcatttaatatctctaaattattctttgctatccgtaatttctctgcagcatcagtttcttttttaagttctttacgaagcctttcattttcagcaataattttttctgtgcctttggtcttggattcatagtgcatgctcaactgatgcccaagatgagctttaagtttttctaattcagccttcaatttttcattttcctgctcaatattagccattttttcactagtcaatattcctgatgcttttttcaactgttcattttctctctggactttttcaactacttttttcattaaaccaatggttttttccagttctgggattgtctttccacttctaccagaccctctaacatggccaagtttccgctgaacttctgctttttctttcttaagaaattcacacatttccttcaaatctctgacttgattctttaatcttggcaaatctttatttgcttgttcaagctgaaatttcagttcaatattttcagatgacaacttcaagttttccttctgaagctcctgttctctctgacaatgatcatctgactctattcctgaaattgaaggcttagaatatgtatcctttgaaaactgtttttctaaagcatgaagtttttcttggaggtatctattttgtaaatgtaaatcttctacaacagaatctcgaggaagagcttggtgggccctcatatacaatatatcattttctaagtcaagatttctcttttttaattcttccaattctttttctgactccaaagctcgtattcccaaaacctgatcaacagtcatgccagttgtttttagtttcctctgcaaagtaagtttctctttatcggctttggcaaaaagatccttcaaagtattcaactgctttgttaaagtaaagacttccccctctttctcttttaacttgtttcgaattccttctattttggcttgccactttttaccttcttcccacctaattaattcttctttagcattcttttctttcataggttttaggtctacttcctccacctttccctctaattggttctctagttttttaactttcctttggagttcttcaattagactttgtttattatctgtcaggggtttgccctgtaatccactggttagtcttttaatttgccttttcagttcatcattctcttgatcaatttcctctttctctctaagtattttattataggctttttgtttcttttgcagttcattatttaagtcattcaaattatcagttagtgagttttctctgtttttacttgttttaagtgcttctttcaattttaaaagattttcatttaaatcttcaacttgtgtctttagctctctagtatgtcgatcaacgatttgttgaacattgagatgggcctctttttgagaagttgcagaaataatacgttcttcagcagctgctgtcatttctgcccggagttctaaaagtgcccgactaagtgctttctgttgtttctccttcaaggctaattggctctttagccgttctactagatttctcattgtagttgttggagctcttgaatttgcttctttttgagcctgaagttcagattttaaacactgtgactccttttgtgactggtccagaagatactttaaatcctctacttccgcttttacttttttcacttcatcttcatggttttcttgaagctgtaatttgatattttcaaattcttttacttttaattcagtgatttctctttgtctctccaaatcttgtgatactttctttagtttgaccaagagtgaggaaagagagtcatcttgttctgctactgtctgttccatctcagccagacgaataaaatgcttgttggtaggaactggagtgggagactgtttcattaaatcccaagccgtttgtttgaatttatttagtgaactatcagcctgtagttctaatctgtgatgaagaatatgaaggtcttcctcatgtttcttcacaatttctctttgctcctctctggctttttctagaagacgttgatacttctttaatacttcttctttttgatttaaccttgcttgcatgtttgcaatggtttgatgagcaattttcaatgtgtggtgagattttggttccatctcttttctgcctagctcagctatgagcttttctctttctgcagtggcaggcaatcgaagcctcagttcattgattactttgtctcttgacagtatattttgttctgctaaccttaaagcagattctttctcttttagtttctcttctagtgatttgcaagttgcccgtgtttctagaattattcgaatgttctccttaattttccttagagcgatctcaagttgatttggaaggggcaaactagggtcagggattgatcctgtagcttcttcaaacttttgtgccgcatttagtatttcattttgctgacggtcaaaaatgtctagttggcgttccaggtcaacttctctttgatcccaggccatttgtctttcttcatgaaacttgttctgttgcacaatttcttcttcaagactgctgattgtacgttcatattcagaaattatgttattcaaatattttatttcttctttatccttgactaattcccgatttagtttaagttcttgaagacgaagttcttctattttcatatgccagttgattaccttttgggctcctttggtatcctttaaagtgcttattaactcttccaggccctttaattttaattccatctccaatgttttgttctccatatttctatgttcttgttgagaatttttcatttcttgcattatcttaagtttgtcattttgtagttgaatcattgttttggagaacttttcctgttgtgccaagggtaaagctccactaaactgtcgtcgtagagactgaattgtttggcgcagatgttttgctctgtttcttccctccaaacgagcataatagagagcctgttctttttcatcaagtttctgctctaagcgcaagttgtaggcctccatcttctgcagtttagatgtaattgactccaacttaccaagagcagtagcctcactcagttgaagagagacattatgttggtgcaacttggcaatgagcgacttttcatcagactgtgcctgatagtctagcagttgcattctgagggactctacttccttgtccctagattgttg

SEQ ID NO: 34 - DNA, 3888 bp, Artificial sequence
  Sequence of expression cassette-CMV-mouse Myo tail-polyA
acgcgtggagctagttattaatagtaatcaattacggggtcattagttcatagcccatatatggagttccgcgttacataacttacggtaaatggcccgcctggctgaccgcccaacgacccccgcccattgacgtcaataatgacgtatgttcccatagtaacgtcaatagggactttccattgacgtcaatgggtggagtatttacggtaaactgcccacttggcagtacatcaagtgtatcatatgccaagtacgccccctattgacgtcaatgacggtaaatggcccgcctggcattatgcccagtacatgaccttatgggactttcctacttggcagtacatctacgtattagtcatcgctattaccatggtgatgcggttttggcagtacatcaatgggcgtggatagcggtttgactcacggggatttccaagtctccaccccattgacgtcaatgggagtttgttttgcaccaaaatcaacgggactttccaaaatgtcgtaacaactccgccccattgacgcaaatgggcggtaggcgtgtacggtgggaggtctatataagcagagctcgtttagtgaaccgtcagatcgcctggagacgccatccacgctgttttgacctccatagaagacaccgggaccgatccagcctccgcggccaccatgttggcagagcaaaatattctgtcaagagacaaagtaatcaatgaactgaggcttcgattgcctgccacggctgatcgagaaaaacttatagctgagctagaaagaaaagagctggagccgaaatctcatcacacaatgaaaattgcccaccaaactattgccaacatgcaggcaaggttaaatcacaaggaagaagtattgaagaaataccagcaccttctggagaaggccagagaggagcaaagagaaattgttaagaagcatgaggaagaccttcatgttcttcatcacaaattagaacaacaggccgataattcactcaataaattcagacagacagctcaggatttacttaagcagtctcctgctccagttcccaccaacaaacatttcattcgtctggccgagatggagcagacagtagcagaacaagatgactctctgtcctcacttttgaccaaactaaagaaagtatcaaaagatttggaaaaacaaaaagaaatcactgagttaaaagtcagagagtttgaaaataccaaactacggctccaagaaactcatgccagtgaggtaaagaaagtgaaagcagaggtagaggacttaaggcatgctctagcccaagcacacaaggactcccagagtttaaagtctgaactccaggctcagaaagaagcaaactccagagctccaacaaccacaatgaggaatcttgtagacaggctaaagagccaactagccttgaaagagaagcaacaaaaggcacttagtcgagccctgttggaacttcggtcggaaatgacagcagcagctgaggaacgtataatcgctgtaacttctcaaaaagaggcaaatctcaatgttcaacaagttgttgagcgccatactagagagctaaagtcacaaattgaagatttaaatgaaaatcttttaaaattgaaagaagctcttaaaacaagtaagaacaaagaaaattcactagctgatgatttaaatgaattaaataatgaactgcaaaaaaagcaaaaagcttataataaaatccttagagagaaagatggaattgatcaagaaaatgatgaactgagaagacagattaaaagactgtccagtggactgcagagcaaaactttgatagataacaagcaaagtttaatcgatgaacttcaaaagaaagttaaaaaacttgaaagccaactggaaagaaaggtggatgacgtagacataaagccggtgaaggaaaagagtagtaaagaagaattaattaggtgggaagaaggtaagaaatggcaaaccaaagtagagggactacgaaacagactaaaggagaaggaaggagaagcccacggcctggcaaagcagctgaataccttaaaggaactttttgccaaagctgataaagagaaacttactttgcagaagaaactgaaaacaacaggaatgactgttgaccaggttttaggagtgcgagctttggaatctgaaaaagagttggaagagctaaaaaagaaaaatctggacctagaaaatgacatattatacatgaggacccagcaggctcttccacgagattctgttgtggaagacttacatttacaaaataaataccttcaagaaaaacttcatactttagaaaaaaaactttcaaaggagaaatattctcagtctttgacttcagaaatagagtcagatgatcactgtcaaaaagaacaagaacttcagaaggaaaatttgaagttgtcatctgaaaacatcgagctgaaatttcaacttgaacaagcaaataaagatttgccaagactaaagaatcaagtgaaagatttgaaggaaatgtgtgaatttcttaagaaaggaaaactggaacttgagcggaagcttggtcaggtcagaggggctggtagaagtgggaagacaatcccagaactagaaaaaaccattgggttaatgaagaaagtagttgaaaaagtccaaagagaaaatgaacaattgaaaaaggcatcaggaatactgactagtgaaaaaatggctactattgaggaagaaaatagaaacttaaaggctgaactagaaaagcttaaagctcactttggacgtcagttgagtatgcagtttgaatctaagaacaaaggtactgagaaaattgttgccgaaaatgaacggcttcggaaagaacttaagaaagaaatagaagcctctgagaaactgcggatagctaagaacaacttagagctggtgaacgacaagatggcagctcaactcgaagaaactgggaagagactacagtttgcagaaagtagagccccacagctggaaggtgctgacagcaagagctggaagtcaattgtggtctcaagagtgtatgagaccaagatgaaagagcttgaaagtgacattgccaaaaagaatcaaagtatcactgaccttaaacagcttgtaagagaagcaacagagagagaacagaaagctaagaaatacactgaagaccttgaacaacagattgagatcctcaaaaatgttcctgaaggtgccgagacagagcaagagcttatacgggaactccagcttcttagattagccaataatcagatggataaagaaagggcagaattaatccatcagatagaaattaacaaggaccaaaccagagctgacagtagcatacctgattctgatcaactaaaggaaaagataaatgacctggagacacaactcagaaagttggagctagaaaagcaacattcgaaggaggaagttaaaaagctgaaaaaagaactggaaaattttgatccttcattttttgaagaaattgaagacctgaagtataattataaggaagaagtgaaaaagaatatcctattagaagagaagctaaaaaaactgtcggaacagtttggatttgaactgcctagtcctcttgctgcttctgaacactcggaagatggagaaagtcctcatagtttccctatttattagagatctacatctcgctttcttgctgtccaatttctattaaaggttcctttgttccctaagtccaactactaaactgggggatattatgaagggccttgagcatctggattctgcctaataaaaaacatttattttcattgcaatgatgtatttaaattatttctgaatattttactaaaaagggaatgtgggaggtcagtgcatttaaaacataaagaaagtaggtaaccacgtgcggaccga

SEQ ID NO: 35 - DNA, 3891 bp, Artificial sequence
  Sequence of expression cassette-CMV-human Myo tail-polyA
acgcgtggagctagttattaatagtaatcaattacggggtcattagttcatagcccatatatggagttccgcgttacataacttacggtaaatggcccgcctggctgaccgcccaacgacccccgcccattgacgtcaataatgacgtatgttcccatagtaacgtcaatagggactttccattgacgtcaatgggtggagtatttacggtaaactgcccacttggcagtacatcaagtgtatcatatgccaagtacgccccctattgacgtcaatgacggtaaatggcccgcctggcattatgcccagtacatgaccttatgggactttcctacttggcagtacatctacgtattagtcatcgctattaccatggtgatgcggttttggcagtacatcaatgggcgtggatagcggtttgactcacggggatttccaagtctccaccccattgacgtcaatgggagtttgttttgcaccaaaatcaacgggactttccaaaatgtcgtaacaactccgccccattgacgcaaatgggcggtaggcgtgtacggtgggaggtctatataagcagagctcgtttagtgaaccgtcagatcgcctggagacgccatccacgctgttttgacctccatagaagacaccgggaccgatccagcctccgcggccaccatgttagcagaacaaaatatactgtcaagagacaaagtaatcaatgaactgaggcttcgattgcctgccactgcagaaagagaaaagctcatagctgagctaggcagaaaagagatggaaccaaaatctcaccacacattgaaaattgctcatcaaaccattgcaaacatgcaagcaaggttaaatcaaaaagaagaagtattaaagaagtatcaacgtcttctagaaaaagccagagaggagcaaagagaaattgtgaagaaacatgaggaagaccttcatattcttcatcacagattagaactacaggctgatagttcactaaataaattcaaacaaacggcttgggatttaatgaaacagtctcccactccagttcctaccaacaagcattttattcgtctggctgagatggaacagacagtagcagaacaagatgactctctttcctcactcttggtcaaactaaagaaagtatcacaagatttggagagacaaagagaaatcactgaattaaaagtaaaagaatttgaaaatatcaaattacagcttcaagaaaaccatgaagatgaagtgaaaaaagtaaaagcggaagtagaggatttaaagtatcttctggaccagtcacaaaaggagtcacagtgtttaaaatctgaacttcaggctcaaaaagaagcaaattcaagagctccaacaactacaatgagaaatctagtagaacggctaaagagccaattagccttgaaggagaaacaacagaaagcacttagtcgggcacttttagaactccgggcagaaatgacagcagctgctgaagaacgtattatttctgcaacttctcaaaaagaggcccatctcaatgttcaacaaatcgttgatcgacatactagagagctaaagacacaagttgaagatttaaatgaaaatcttttaaaattgaaagaagcacttaaaacaagtaaaaacagagaaaactcactaactgataatttgaatgacttaaataatgaactgcaaaagaaacaaaaagcctataataaaatacttagagagaaagaggaaattgatcaagagaatgatgaactgaaaaggcaaattaaaagactaaccagtggattacagggcaaacccctgacagataataaacaaagtctaattgaagaactccaaaggaaagttaaaaaactagagaaccaattagagggaaaggtggaggaagtagacctaaaacctatgaaagaaaagaatgctaaagaagaattaattaggtgggaagaaggtaaaaagtggcaagccaaaatagaaggaattcgaaacaagttaaaagagaaagagggggaagtctttactttaacaaagcagttgaatactttgaaggatctttttgccaaagccgataaagagaaacttactttgcagaggaaactaaaaacaactggcatgactgttgatcaggttttgggaatacgagctttggagtcagaaaaagaattggaagaattaaaaaagagaaatcttgacttagaaaatgatatattgtatatgagggcccaccaagctcttcctcgagattctgttgtagaagatttacatttacaaaatagatacctccaagaaaaacttcatgctttagaaaaacagttttcaaaggatacatattctaagccttcaatttcaggaatagagtcagatgatcattgtcagagagaacaggagcttcagaaggaaaacttgaagttgtcatctgaaaatattgaactgaaatttcagcttgaacaagcaaataaagatttgccaagattaaagaatcaagtcagagatttgaaggaaatgtgtgaatttcttaagaaagaaaaagcagaagttcagcggaaacttggccatgttagagggtctggtagaagtggaaagacaatcccagaactggaaaaaaccattggtttaatgaaaaaagtagttgaaaaagtccagagagaaaatgaacagttgaaaaaagcatcaggaatattgactagtgaaaaaatggctaatattgagcaggaaaatgaaaaattgaaggctgaattagaaaaacttaaagctcatcttgggcatcagttgagcatgcactatgaatccaagaccaaaggcacagaaaaaattattgctgaaaatgaaaggcttcgtaaagaacttaaaaaagaaactgatgctgcagagaaattacggatagcaaagaataatttagagatattaaatgagaagatgacagttcaactagaagagactggtaagagattgcagtttgcagaaagcagaggtccacagcttgaaggtgctgacagtaagagctggaaatccattgtggttacaagaatgtatgaaaccaagttaaaagaattggaaactgatattgccaaaaaaaatcaaagcattactgaccttaaacagcttgtaaaagaagcaacagagagagaacaaaaagttaacaaatacaatgaagaccttgaacaacagattaagattcttaaacatgttcctgaaggtgctgagacagagcaaggccttaaacgggagcttcaagttcttagattagctaatcatcagctggataaagagaaagcagaattaatccatcagatagaagctaacaaggaccaaagtggagctgaaagcaccatacctgatgctgatcaactaaaggaaaaaataaaagatctagagacacagctcaaaatgtcagatctagaaaagcagcatttgaaggaggaaataaagaagctgaaaaaagaactggaaaattttgatccttcattttttgaagaaattgaagatcttaagtataattacaaggaagaagtgaagaagaatattctcttagaagagaaggtaaaaaaactttcagaacaattgggagttgaattaactagccctgttgctgcttctgaagagtttgaagatgaagaagaaagtcctgttaatttccccatttactaaagatctacatctcgctttcttgctgtccaatttctattaaaggttcctttgttccctaagtccaactactaaactgggggatattatgaagggccttgagcatctggattctgcctaataaaaaacatttattttcattgcaatgatgtatttaaattatttctgaatattttactaaaaagggaatgtgggaggtcagtgcatttaaaacataaagaaagtaggtaaccacgtgcggaccga

SEQ ID NO: 36 - DNA, 1818 bp, Artificial sequence
  Sequence of expression cassette-CMV-mouse DSD-polyA
acgcgtggagctagttattaatagtaatcaattacggggtcattagttcatagcccatatatggagttccgcgttacataacttacggtaaatggcccgcctggctgaccgcccaacgacccccgcccattgacgtcaataatgacgtatgttcccatagtaacgtcaatagggactttccattgacgtcaatgggtggagtatttacggtaaactgcccacttggcagtacatcaagtgtatcatatgccaagtacgccccctattgacgtcaatgacggtaaatggcccgcctggcattatgcccagtacatgaccttatgggactttcctacttggcagtacatctacgtattagtcatcgctattaccatggtgatgcggttttggcagtacatcaatgggcgtggatagcggtttgactcacggggatttccaagtctccaccccattgacgtcaatgggagtttgttttgcaccaaaatcaacgggactttccaaaatgtcgtaacaactccgccccattgacgcaaatgggcggtaggcgtgtacggtgggaggtctatataagcagagctcgtttagtgaaccgtcagatcgcctggagacgccatccacgctgttttgacctccatagaagacaccgggaccgatccagcctccgcggccaccatggatttacttaagcagtctcctgctccagttcccaccaacaaacatttcattcgtctggccgagatggagcagacagtagcagaacaagatgactctctgtcctcacttttgaccaaactaaagaaagtatcaaaagatttggaaaaacaaaaagaaatcactgagttaaaagtcagagagtttgaaaataccaaactacggctccaagaaactcatgccagtgaggtaaagaaagtgaaagcagaggtagaggacttaaggcatgctctagcccaagcacacaaggactcccagagtttaaagtctgaactccaggctcagaaagaagcaaactccagagctccaacaaccacaatgaggaatcttgtagacaggctaaagagccaactagccttgaaagagaagcaacaaaaggcacttagtcgagccctgttggaacttcggtcggaaatgacagcagcagctgaggaacgtataatcgctgtaacttctcaaaaagaggcaaatctcaatgttcaacaagttgttgagcgccatactagagagctaaagtcacaaattgaagatttaaatgaaaatcttttaaaattgaaagaagctcttaaaacaagtaagaacaaagaaaattcactagctgatgatttaaatgaattaaataatgaactgcaaaaaaagcaaaaagcttataataaaatccttagagagaaagatggaattgatcaagaaaatgatgaactgagaagacagattaaaagactgtccagtggactgcagagcaaaactttgatagataacaagcaaagtttaatcgatgaacttcaaaagaaagttaaaaaacttgaaagccaactggaaagaaaggtggatgacgtagacataaagccggtgaaggaaaagtagagatctacatctcgctttcttgctgtccaatttctattaaaggttcctttgttccctaagtccaactactaaactgggggatattatgaagggccttgagcatctggattctgcctaataaaaaacatttattttcattgcaatgatgtatttaaattatttctgaatattttactaaaaagggaatgtgggaggtcagtgcatttaaaacataaagaaagtaggtaaccacgtgcggaccga

SEQ ID NO: 37 - DNA, 1818 bp, Artificial sequence
  Sequence of expression cassette-CMV-human DSD-polyA
acgcgtggagctagttattaatagtaatcaattacggggtcattagttcatagcccatatatggagttccgcgttacataacttacggtaaatggcccgcctggctgaccgcccaacgacccccgcccattgacgtcaataatgacgtatgttcccatagtaacgtcaatagggactttccattgacgtcaatgggtggagtatttacggtaaactgcccacttggcagtacatcaagtgtatcatatgccaagtacgccccctattgacgtcaatgacggtaaatggcccgcctggcattatgcccagtacatgaccttatgggactttcctacttggcagtacatctacgtattagtcatcgctattaccatggtgatgcggttttggcagtacatcaatgggcgtggatagcggtttgactcacggggatttccaagtctccaccccattgacgtcaatgggagtttgttttgcaccaaaatcaacgggactttccaaaatgtcgtaacaactccgccccattgacgcaaatgggcggtaggcgtgtacggtgggaggtctatataagcagagctcgtttagtgaaccgtcagatcgcctggagacgccatccacgctgttttgacctccatagaagacaccgggaccgatccagcctccgcggccaccatggatttaatgaaacagtctcccactccagttcctaccaacaagcattttattcgtctggctgagatggaacagacagtagcagaacaagatgactctctttcctcactcttggtcaaactaaagaaagtatcacaagatttggagagacaaagagaaatcactgaattaaaagtaaaagaatttgaaaatatcaaattacagcttcaagaaaaccatgaagatgaagtgaaaaaagtaaaagcggaagtagaggatttaaagtatcttctggaccagtcacaaaaggagtcacagtgtttaaaatctgaacttcaggctcaaaaagaagcaaattcaagagctccaacaactacaatgagaaatctagtagaacggctaaagagccaattagccttgaaggagaaacaacagaaagcacttagtcgggcacttttagaactccgggcagaaatgacagcagctgctgaagaacgtattatttctgcaacttctcaaaaagaggcccatctcaatgttcaacaaatcgttgatcgacatactagagagctaaagacacaagttgaagatttaaatgaaaatcttttaaaattgaaagaagcacttaaaacaagtaaaaacagagaaaactcactaactgataatttgaatgacttaaataatgaactgcaaaagaaacaaaaagcctataataaaatacttagagagaaagaggaaattgatcaagagaatgatgaactgaaaaggcaaattaaaagactaaccagtggattacagggcaaacccctgacagataataaacaaagtctaattgaagaactccaaaggaaagttaaaaaactagagaaccaattagagggaaaggtggaggaagtagacctaaaacctatgaaagaaaagtagagatctacatctcgctttcttgctgtccaatttctattaaaggttcctttgttccctaagtccaactactaaactgggggatattatgaagggccttgagcatctggattctgcctaataaaaaacatttattttcattgcaatgatgtatttaaattatttctgaatattttactaaaaagggaatgtgggaggtcagtgcatttaaaacataaagaaagtaggtaaccacgtgcggaccga

SEQ ID NO: 38 - DNA, 4842 bp, Artificial sequence
  Sequence of expression cassette-CMV-mouse C-terminal-polyA
acgcgtggagctagttattaatagtaatcaattacggggtcattagttcatagcccatatatggagttccgcgttacataacttacggtaaatggcccgcctggctgaccgcccaacgacccccgcccattgacgtcaataatgacgtatgttcccatagtaacgtcaatagggactttccattgacgtcaatgggtggagtatttacggtaaactgcccacttggcagtacatcaagtgtatcatatgccaagtacgccccctattgacgtcaatgacggtaaatggcccgcctggcattatgcccagtacatgaccttatgggactttcctacttggcagtacatctacgtattagtcatcgctattaccatggtgatgcggttttggcagtacatcaatgggcgtggatagcggtttgactcacggggatttccaagtctccaccccattgacgtcaatgggagtttgttttgcaccaaaatcaacgggactttccaaaatgtcgtaacaactccgccccattgacgcaaatgggcggtaggcgtgtacggtgggaggtctatataagcagagctcgtttagtgaaccgtcagatcgcctggagacgccatccacgctgttttgacctccatagaagacaccgggaccgatccagcctccgcggccaccatgcaacaacagtccagggaaaaggaagtggaatccctcagaacgcagctgctggacttccaggcacaatctgacgaaaaggctctaattgccaaattgcaccaacatgttgtctctcttcaaattagtgaggccactgccctcggtaagttagagtcagttacgtccaaactccagaagatggaagcctacaatttgcgcttagaacagaaactggatgaaaaagagcaggcgctctactatgctcgtttggaaggtagaaacagagcaaaacacctgcgccaaaccattcagtcgcttcgaagacagttcagtggagctctacccttagcacagcaggaaaagttctccaaaacgatgattcagttgcaaaatgacaaacttaagataatgcaagaaatgaagaattcgcaacaggaacacagaaatatggaaaacaaaacactggagttggaattaaaattaaaaggcttagaagaattgatcagtactttaaaggatgccaggggagcccagaaggtaatcaattggcatgtgaaaatagaagaacttcgcctccaagaacttaagctaaatagagaactagtcaagggtaaagaagaaatcaaatatttgaataatatcatctctgaatatgagcatacaatcaacagtctagaggaagaaattgttcagcaaagcaagttccatgaagaaagacagatggcttgggatcaaagagaagttgagctggaacgccagttagacatttttgatcatcagcaaaatgaaatactcagtgcagcacaaaagtttgaagactctacaggatcaatgccagaccccagcttgcctcttccaaaccaacttgaaattgctctaagaaaaattaaggagaatattcaagtaattcttaaaacacaagcaacttgcaagtcactagaagagaaactaaaagaaaaagaatctgctttacggttggcagagcaaaatattctgtcaagagacaaagtaatcaatgaactgaggcttcgattgcctgccacggctgatcgagaaaaacttatagctgagctagaaagaaaagagctggagccgaaatctcatcacacaatgaaaattgcccaccaaactattgccaacatgcaggcaaggttaaatcacaaggaagaagtattgaagaaataccagcaccttctggagaaggccagagaggagcaaagagaaattgttaagaagcatgaggaagaccttcatgttcttcatcacaaattagaacaacaggccgataattcactcaataaattcagacagacagctcaggatttacttaagcagtctcctgctccagttcccaccaacaaacatttcattcgtctggccgagatggagcagacagtagcagaacaagatgactctctgtcctcacttttgaccaaactaaagaaagtatcaaaagatttggaaaaacaaaaagaaatcactgagttaaaagtcagagagtttgaaaataccaaactacggctccaagaaactcatgccagtgaggtaaagaaagtgaaagcagaggtagaggacttaaggcatgctctagcccaagcacacaaggactcccagagtttaaagtctgaactccaggctcagaaagaagcaaactccagagctccaacaaccacaatgaggaatcttgtagacaggctaaagagccaactagccttgaaagagaagcaacaaaaggcacttagtcgagccctgttggaacttcggtcggaaatgacagcagcagctgaggaacgtataatcgctgtaacttctcaaaaagaggcaaatctcaatgttcaacaagttgttgagcgccatactagagagctaaagtcacaaattgaagatttaaatgaaaatcttttaaaattgaaagaagctcttaaaacaagtaagaacaaagaaaattcactagctgatgatttaaatgaattaaataatgaactgcaaaaaaagcaaaaagcttataataaaatccttagagagaaagatggaattgatcaagaaaatgatgaactgagaagacagattaaaagactgtccagtggactgcagagcaaaactttgatagataacaagcaaagtttaatcgatgaacttcaaaagaaagttaaaaaacttgaaagccaactggaaagaaaggtggatgacgtagacataaagccggtgaaggaaaagagtagtaaagaagaattaattaggtgggaagaaggtaagaaatggcaaaccaaagtagagggactacgaaacagactaaaggagaaggaaggagaagcccacggcctggcaaagcagctgaataccttaaaggaactttttgccaaagctgataaagagaaacttactttgcagaagaaactgaaaacaacaggaatgactgttgaccaggttttaggagtgcgagctttggaatctgaaaaagagttggaagagctaaaaaagaaaaatctggacctagaaaatgacatattatacatgaggacccagcaggctcttccacgagattctgttgtggaagacttacatttacaaaataaataccttcaagaaaaacttcatactttagaaaaaaaactttcaaaggagaaatattctcagtctttgacttcagaaatagagtcagatgatcactgtcaaaaagaacaagaacttcagaaggaaaatttgaagttgtcatctgaaaacatcgagctgaaatttcaacttgaacaagcaaataaagatttgccaagactaaagaatcaagtgaaagatttgaaggaaatgtgtgaatttcttaagaaaggaaaactggaacttgagcggaagcttggtcaggtcagaggggctggtagaagtgggaagacaatcccagaactagaaaaaaccattgggttaatgaagaaagtagttgaaaaagtccaaagagaaaatgaacaattgaaaaaggcatcaggaatactgactagtgaaaaaatggctactattgaggaagaaaatagaaacttaaaggctgaactagaaaagcttaaagctcactttggacgtcagttgagtatgcagtttgaatctaagaacaaaggtactgagaaaattgttgccgaaaatgaacggcttcggaaagaacttaagaaagaaatagaagcctctgagaaactgcggatagctaagaacaacttagagctggtgaacgacaagatggcagctcaactcgaagaaactgggaagagactacagtttgcagaaagtagagccccacagctggaaggtgctgacagcaagagctggaagtcaattgtggtctcaagagtgtatgagaccaagatgaaagagcttgaaagtgacattgccaaaaagaatcaaagtatcactgaccttaaacagcttgtaagagaagcaacagagagagaacagaaagctaagaaatacactgaagaccttgaacaacagattgagatcctcaaaaatgttcctgaaggtgccgagacagagcaagagcttatacgggaactccagcttcttagattagccaataatcagatggataaagaaagggcagaattaatccatcagatagaaattaacaaggaccaaaccagagctgacagtagcatacctgattctgatcaactaaaggaaaagataaatgacctggagacacaactcagaaagttggagctagaaaagcaacattcgaaggaggaagttaaaaagctgaaaaaagaactggaaaattttgatccttcattttttgaagaaattgaagacctgaagtataattataaggaagaagtgaaaaagaatatcctattagaagagaagctaaaaaaactgtcggaacagtttggatttgaactgcctagtcctcttgctgcttctgaacactcggaagatggagaaagtcctcatagtttccctatttattagagatctacatctcgctttcttgctgtccaatttctattaaaggttcctttgttccctaagtccaactactaaactgggggatattatgaagggccttgagcatctggattctgcctaataaaaaacatttattttcattgcaatgatgtatttaaattatttctgaatattttactaaaaagggaatgtgggaggtcagtgcatttaaaacataaagaaagtaggtaaccacgtgcggaccga

SEQ ID NO: 39 - DNA, 4842 bp, Artificial sequence
  Sequence of expression cassette-CMV-human C-terminal-polyA
acgcgtggagctagttattaatagtaatcaattacggggtcattagttcatagcccatatatggagttccgcgttacataacttacggtaaatggcccgcctggctgaccgcccaacgacccccgcccattgacgtcaataatgacgtatgttcccatagtaacgtcaatagggactttccattgacgtcaatgggtggagtatttacggtaaactgcccacttggcagtacatcaagtgtatcatatgccaagtacgccccctattgacgtcaatgacggtaaatggcccgcctggcattatgcccagtacatgaccttatgggactttcctacttggcagtacatctacgtattagtcatcgctattaccatggtgatgcggttttggcagtacatcaatgggcgtggatagcggtttgactcacggggatttccaagtctccaccccattgacgtcaatgggagtttgttttgcaccaaaatcaacgggactttccaaaatgtcgtaacaactccgccccattgacgcaaatgggcggtaggcgtgtacggtgggaggtctatataagcagagctcgtttagtgaaccgtcagatcgcctggagacgccatccacgctgttttgacctccatagaagacaccgggaccgatccagcctccgcggccaccatgcaacaatctagggacaaggaagtagagtccctcagaatgcaactgctagactatcaggcacagtctgatgaaaagtcgctcattgccaagttgcaccaacataatgtctctcttcaactgagtgaggctactgctcttggtaagttggagtcaattacatctaaactgcagaagatggaggcctacaacttgcgcttagagcagaaacttgatgaaaaagaacaggctctctattatgctcgtttggagggaagaaacagagcaaaacatctgcgccaaacaattcagtctctacgacgacagtttagtggagctttacccttggcacaacaggaaaagttctccaaaacaatgattcaactacaaaatgacaaacttaagataatgcaagaaatgaaaaattctcaacaagaacatagaaatatggagaacaaaacattggagatggaattaaaattaaagggcctggaagagttaataagcactttaaaggataccaaaggagcccaaaaggtaatcaactggcatatgaaaatagaagaacttcgtcttcaagaacttaaactaaatcgggaattagtcaaggataaagaagaaataaaatatttgaataacataatttctgaatatgaacgtacaatcagcagtcttgaagaagaaattgtgcaacagaacaagtttcatgaagaaagacaaatggcctgggatcaaagagaagttgacctggaacgccaactagacatttttgaccgtcagcaaaatgaaatactaaatgcggcacaaaagtttgaagaagctacaggatcaatccctgaccctagtttgccccttccaaatcaacttgagatcgctctaaggaaaattaaggagaacattcgaataattctagaaacacgggcaacttgcaaatcactagaagagaaactaaaagagaaagaatctgctttaaggttagcagaacaaaatatactgtcaagagacaaagtaatcaatgaactgaggcttcgattgcctgccactgcagaaagagaaaagctcatagctgagctaggcagaaaagagatggaaccaaaatctcaccacacattgaaaattgctcatcaaaccattgcaaacatgcaagcaaggttaaatcaaaaagaagaagtattaaagaagtatcaacgtcttctagaaaaagccagagaggagcaaagagaaattgtgaagaaacatgaggaagaccttcatattcttcatcacagattagaactacaggctgatagttcactaaataaattcaaacaaacggcttgggatttaatgaaacagtctcccactccagttcctaccaacaagcattttattcgtctggctgagatggaacagacagtagcagaacaagatgactctctttcctcactcttggtcaaactaaagaaagtatcacaagatttggagagacaaagagaaatcactgaattaaaagtaaaagaatttgaaaatatcaaattacagcttcaagaaaaccatgaagatgaagtgaaaaaagtaaaagcggaagtagaggatttaaagtatcttctggaccagtcacaaaaggagtcacagtgtttaaaatctgaacttcaggctcaaaaagaagcaaattcaagagctccaacaactacaatgagaaatctagtagaacggctaaagagccaattagccttgaaggagaaacaacagaaagcacttagtcgggcacttttagaactccgggcagaaatgacagcagctgctgaagaacgtattatttctgcaacttctcaaaaagaggcccatctcaatgttcaacaaatcgttgatcgacatactagagagctaaagacacaagttgaagatttaaatgaaaatcttttaaaattgaaagaagcacttaaaacaagtaaaaacagagaaaactcactaactgataatttgaatgacttaaataatgaactgcaaaagaaacaaaaagcctataataaaatacttagagagaaagaggaaattgatcaagagaatgatgaactgaaaaggcaaattaaaagactaaccagtggattacagggcaaacccctgacagataataaacaaagtctaattgaagaactccaaaggaaagttaaaaaactagagaaccaattagagggaaaggtggaggaagtagacctaaaacctatgaaagaaaagaatgctaaagaagaattaattaggtgggaagaaggtaaaaagtggcaagccaaaatagaaggaattcgaaacaagttaaaagagaaagagggggaagtctttactttaacaaagcagttgaatactttgaaggatctttttgccaaagccgataaagagaaacttactttgcagaggaaactaaaaacaactggcatgactgttgatcaggttttgggaatacgagctttggagtcagaaaaagaattggaagaattaaaaaagagaaatcttgacttagaaaatgatatattgtatatgagggcccaccaagctcttcctcgagattctgttgtagaagatttacatttacaaaatagatacctccaagaaaaacttcatgctttagaaaaacagttttcaaaggatacatattctaagccttcaatttcaggaatagagtcagatgatcattgtcagagagaacaggagcttcagaaggaaaacttgaagttgtcatctgaaaatattgaactgaaatttcagcttgaacaagcaaataaagatttgccaagattaaagaatcaagtcagagatttgaaggaaatgtgtgaatttcttaagaaagaaaaagcagaagttcagcggaaacttggccatgttagagggtctggtagaagtggaaagacaatcccagaactggaaaaaaccattggtttaatgaaaaaagtagttgaaaaagtccagagagaaaatgaacagttgaaaaaagcatcaggaatattgactagtgaaaaaatggctaatattgagcaggaaaatgaaaaattgaaggctgaattagaaaaacttaaagctcatcttgggcatcagttgagcatgcactatgaatccaagaccaaaggcacagaaaaaattattgctgaaaatgaaaggcttcgtaaagaacttaaaaaagaaactgatgctgcagagaaattacggatagcaaagaataatttagagatattaaatgagaagatgacagttcaactagaagagactggtaagagattgcagtttgcagaaagcagaggtccacagcttgaaggtgctgacagtaagagctggaaatccattgtggttacaagaatgtatgaaaccaagttaaaagaattggaaactgatattgccaaaaaaaatcaaagcattactgaccttaaacagcttgtaaaagaagcaacagagagagaacaaaaagttaacaaatacaatgaagaccttgaacaacagattaagattcttaaacatgttcctgaaggtgctgagacagagcaaggccttaaacgggagcttcaagttcttagattagctaatcatcagctggataaagagaaagcagaattaatccatcagatagaagctaacaaggaccaaagtggagctgaaagcaccatacctgatgctgatcaactaaaggaaaaaataaaagatctagagacacagctcaaaatgtcagatctagaaaagcagcatttgaaggaggaaataaagaagctgaaaaaagaactggaaaattttgatccttcattttttgaagaaattgaagatcttaagtataattacaaggaagaagtgaagaagaatattctcttagaagagaaggtaaaaaaactttcagaacaattgggagttgaattaactagccctgttgctgcttctgaagagtttgaagatgaagaagaaagtcctgttaatttccccatttactaaagatctacatctcgctttcttgctgtccaatttctattaaaggttcctttgttccctaagtccaactactaaactgggggatattatgaagggccttgagcatctggattctgcctaataaaaaacatttattttcattgcaatgatgtatttaaattatttctgaatattttactaaaaagggaatgtgggaggtcagtgcatttaaaacataaagaaagtaggtaaccacgtgcggaccga

SEQ ID NO: 40 - DNA, 4178 bp, Artificial sequence
  Sequence of mouse Myo tail expression vector
ggcagctgcgcgctcgctcgctcactgaggccgcccgggcaaagcccgggcgtcgggcgacctttggtcgcccggcctcagtgagcgagcgagcgcgcagagagggagtggccaactccatcactaggggttcctgcggccgcacgcgtggagctagttattaatagtaatcaattacggggtcattagttcatagcccatatatggagttccgcgttacataacttacggtaaatggcccgcctggctgaccgcccaacgacccccgcccattgacgtcaataatgacgtatgttcccatagtaacgtcaatagggactttccattgacgtcaatgggtggagtatttacggtaaactgcccacttggcagtacatcaagtgtatcatatgccaagtacgccccctattgacgtcaatgacggtaaatggcccgcctggcattatgcccagtacatgaccttatgggactttcctacttggcagtacatctacgtattagtcatcgctattaccatggtgatgcggttttggcagtacatcaatgggcgtggatagcggtttgactcacggggatttccaagtctccaccccattgacgtcaatgggagtttgttttgcaccaaaatcaacgggactttccaaaatgtcgtaacaactccgccccattgacgcaaatgggcggtaggcgtgtacggtgggaggtctatataagcagagctcgtttagtgaaccgtcagatcgcctggagacgccatccacgctgttttgacctccatagaagacaccgggaccgatccagcctccgcggccaccatgttggcagagcaaaatattctgtcaagagacaaagtaatcaatgaactgaggcttcgattgcctgccacggctgatcgagaaaaacttatagctgagctagaaagaaaagagctggagccgaaatctcatcacacaatgaaaattgcccaccaaactattgccaacatgcaggcaaggttaaatcacaaggaagaagtattgaagaaataccagcaccttctggagaaggccagagaggagcaaagagaaattgttaagaagcatgaggaagaccttcatgttcttcatcacaaattagaacaacaggccgataattcactcaataaattcagacagacagctcaggatttacttaagcagtctcctgctccagttcccaccaacaaacatttcattcgtctggccgagatggagcagacagtagcagaacaagatgactctctgtcctcacttttgaccaaactaaagaaagtatcaaaagatttggaaaaacaaaaagaaatcactgagttaaaagtcagagagtttgaaaataccaaactacggctccaagaaactcatgccagtgaggtaaagaaagtgaaagcagaggtagaggacttaaggcatgctctagcccaagcacacaaggactcccagagtttaaagtctgaactccaggctcagaaagaagcaaactccagagctccaacaaccacaatgaggaatcttgtagacaggctaaagagccaactagccttgaaagagaagcaacaaaaggcacttagtcgagccctgttggaacttcggtcggaaatgacagcagcagctgaggaacgtataatcgctgtaacttctcaaaaagaggcaaatctcaatgttcaacaagttgttgagcgccatactagagagctaaagtcacaaattgaagatttaaatgaaaatcttttaaaattgaaagaagctcttaaaacaagtaagaacaaagaaaattcactagctgatgatttaaatgaattaaataatgaactgcaaaaaaagcaaaaagcttataataaaatccttagagagaaagatggaattgatcaagaaaatgatgaactgagaagacagattaaaagactgtccagtggactgcagagcaaaactttgatagataacaagcaaagtttaatcgatgaacttcaaaagaaagttaaaaaacttgaaagccaactggaaagaaaggtggatgacgtagacataaagccggtgaaggaaaagagtagtaaagaagaattaattaggtgggaagaaggtaagaaatggcaaaccaaagtagagggactacgaaacagactaaaggagaaggaaggagaagcccacggcctggcaaagcagctgaataccttaaaggaactttttgccaaagctgataaagagaaacttactttgcagaagaaactgaaaacaacaggaatgactgttgaccaggttttaggagtgcgagctttggaatctgaaaaagagttggaagagctaaaaaagaaaaatctggacctagaaaatgacatattatacatgaggacccagcaggctcttccacgagattctgttgtggaagacttacatttacaaaataaataccttcaagaaaaacttcatactttagaaaaaaaactttcaaaggagaaatattctcagtctttgacttcagaaatagagtcagatgatcactgtcaaaaagaacaagaacttcagaaggaaaatttgaagttgtcatctgaaaacatcgagctgaaatttcaacttgaacaagcaaataaagatttgccaagactaaagaatcaagtgaaagatttgaaggaaatgtgtgaatttcttaagaaaggaaaactggaacttgagcggaagcttggtcaggtcagaggggctggtagaagtgggaagacaatcccagaactagaaaaaaccattgggttaatgaagaaagtagttgaaaaagtccaaagagaaaatgaacaattgaaaaaggcatcaggaatactgactagtgaaaaaatggctactattgaggaagaaaatagaaacttaaaggctgaactagaaaagcttaaagctcactttggacgtcagttgagtatgcagtttgaatctaagaacaaaggtactgagaaaattgttgccgaaaatgaacggcttcggaaagaacttaagaaagaaatagaagcctctgagaaactgcggatagctaagaacaacttagagctggtgaacgacaagatggcagctcaactcgaagaaactgggaagagactacagtttgcagaaagtagagccccacagctggaaggtgctgacagcaagagctggaagtcaattgtggtctcaagagtgtatgagaccaagatgaaagagcttgaaagtgacattgccaaaaagaatcaaagtatcactgaccttaaacagcttgtaagagaagcaacagagagagaacagaaagctaagaaatacactgaagaccttgaacaacagattgagatcctcaaaaatgttcctgaaggtgccgagacagagcaagagcttatacgggaactccagcttcttagattagccaataatcagatggataaagaaagggcagaattaatccatcagatagaaattaacaaggaccaaaccagagctgacagtagcatacctgattctgatcaactaaaggaaaagataaatgacctggagacacaactcagaaagttggagctagaaaagcaacattcgaaggaggaagttaaaaagctgaaaaaagaactggaaaattttgatccttcattttttgaagaaattgaagacctgaagtataattataaggaagaagtgaaaaagaatatcctattagaagagaagctaaaaaaactgtcggaacagtttggatttgaactgcctagtcctcttgctgcttctgaacactcggaagatggagaaagtcctcatagtttccctatttattagagatctacatctcgctttcttgctgtccaatttctattaaaggttcctttgttccctaagtccaactactaaactgggggatattatgaagggccttgagcatctggattctgcctaataaaaaacatttattttcattgcaatgatgtatttaaattatttctgaatattttactaaaaagggaatgtgggaggtcagtgcatttaaaacataaagaaagtaggtaaccacgtgcggaccgagcggccgcaggaacccctagtgatggagttggccactccctctctgcgcgctcgctcgctcactgaggccgggcgaccaaaggtcgcccgacgcccgggctttgcccgggcggcctcagtgagcgagcgagcgcgcagctgcctgca

SEQ ID NO: 41 - DNA, 4181 bp, Artificial sequence
  Sequence of human Myo tail expression vector
ggcagctgcgcgctcgctcgctcactgaggccgcccgggcaaagcccgggcgtcgggcgacctttggtcgcccggcctcagtgagcgagcgagcgcgcagagagggagtggccaactccatcactaggggttcctgcggccgcacgcgtggagctagttattaatagtaatcaattacggggtcattagttcatagcccatatatggagttccgcgttacataacttacggtaaatggcccgcctggctgaccgcccaacgacccccgcccattgacgtcaataatgacgtatgttcccatagtaacgtcaatagggactttccattgacgtcaatgggtggagtatttacggtaaactgcccacttggcagtacatcaagtgtatcatatgccaagtacgccccctattgacgtcaatgacggtaaatggcccgcctggcattatgcccagtacatgaccttatgggactttcctacttggcagtacatctacgtattagtcatcgctattaccatggtgatgcggttttggcagtacatcaatgggcgtggatagcggtttgactcacggggatttccaagtctccaccccattgacgtcaatgggagtttgttttgcaccaaaatcaacgggactttccaaaatgtcgtaacaactccgccccattgacgcaaatgggcggtaggcgtgtacggtgggaggtctatataagcagagctcgtttagtgaaccgtcagatcgcctggagacgccatccacgctgttttgacctccatagaagacaccgggaccgatccagcctccgcggccaccatgttagcagaacaaaatatactgtcaagagacaaagtaatcaatgaactgaggcttcgattgcctgccactgcagaaagagaaaagctcatagctgagctaggcagaaaagagatggaaccaaaatctcaccacacattgaaaattgctcatcaaaccattgcaaacatgcaagcaaggttaaatcaaaaagaagaagtattaaagaagtatcaacgtcttctagaaaaagccagagaggagcaaagagaaattgtgaagaaacatgaggaagaccttcatattcttcatcacagattagaactacaggctgatagttcactaaataaattcaaacaaacggcttgggatttaatgaaacagtctcccactccagttcctaccaacaagcattttattcgtctggctgagatggaacagacagtagcagaacaagatgactctctttcctcactcttggtcaaactaaagaaagtatcacaagatttggagagacaaagagaaatcactgaattaaaagtaaaagaatttgaaaatatcaaattacagcttcaagaaaaccatgaagatgaagtgaaaaaagtaaaagcggaagtagaggatttaaagtatcttctggaccagtcacaaaaggagtcacagtgtttaaaatctgaacttcaggctcaaaaagaagcaaattcaagagctccaacaactacaatgagaaatctagtagaacggctaaagagccaattagccttgaaggagaaacaacagaaagcacttagtcgggcacttttagaactccgggcagaaatgacagcagctgctgaagaacgtattatttctgcaacttctcaaaaagaggcccatctcaatgttcaacaaatcgttgatcgacatactagagagctaaagacacaagttgaagatttaaatgaaaatcttttaaaattgaaagaagcacttaaaacaagtaaaaacagagaaaactcactaactgataatttgaatgacttaaataatgaactgcaaaagaaacaaaaagcctataataaaatacttagagagaaagaggaaattgatcaagagaatgatgaactgaaaaggcaaattaaaagactaaccagtggattacagggcaaacccctgacagataataaacaaagtctaattgaagaactccaaaggaaagttaaaaaactagagaaccaattagagggaaaggtggaggaagtagacctaaaacctatgaaagaaaagaatgctaaagaagaattaattaggtgggaagaaggtaaaaagtggcaagccaaaatagaaggaattcgaaacaagttaaaagagaaagagggggaagtctttactttaacaaagcagttgaatactttgaaggatctttttgccaaagccgataaagagaaacttactttgcagaggaaactaaaaacaactggcatgactgttgatcaggttttgggaatacgagctttggagtcagaaaaagaattggaagaattaaaaaagagaaatcttgacttagaaaatgatatattgtatatgagggcccaccaagctcttcctcgagattctgttgtagaagatttacatttacaaaatagatacctccaagaaaaacttcatgctttagaaaaacagttttcaaaggatacatattctaagccttcaatttcaggaatagagtcagatgatcattgtcagagagaacaggagcttcagaaggaaaacttgaagttgtcatctgaaaatattgaactgaaatttcagcttgaacaagcaaataaagatttgccaagattaaagaatcaagtcagagatttgaaggaaatgtgtgaatttcttaagaaagaaaaagcagaagttcagcggaaacttggccatgttagagggtctggtagaagtggaaagacaatcccagaactggaaaaaaccattggtttaatgaaaaaagtagttgaaaaagtccagagagaaaatgaacagttgaaaaaagcatcaggaatattgactagtgaaaaaatggctaatattgagcaggaaaatgaaaaattgaaggctgaattagaaaaacttaaagctcatcttgggcatcagttgagcatgcactatgaatccaagaccaaaggcacagaaaaaattattgctgaaaatgaaaggcttcgtaaagaacttaaaaaagaaactgatgctgcagagaaattacggatagcaaagaataatttagagatattaaatgagaagatgacagttcaactagaagagactggtaagagattgcagtttgcagaaagcagaggtccacagcttgaaggtgctgacagtaagagctggaaatccattgtggttacaagaatgtatgaaaccaagttaaaagaattggaaactgatattgccaaaaaaaatcaaagcattactgaccttaaacagcttgtaaaagaagcaacagagagagaacaaaaagttaacaaatacaatgaagaccttgaacaacagattaagattcttaaacatgttcctgaaggtgctgagacagagcaaggccttaaacgggagcttcaagttcttagattagctaatcatcagctggataaagagaaagcagaattaatccatcagatagaagctaacaaggaccaaagtggagctgaaagcaccatacctgatgctgatcaactaaaggaaaaaataaaagatctagagacacagctcaaaatgtcagatctagaaaagcagcatttgaaggaggaaataaagaagctgaaaaaagaactggaaaattttgatccttcattttttgaagaaattgaagatcttaagtataattacaaggaagaagtgaagaagaatattctcttagaagagaaggtaaaaaaactttcagaacaattgggagttgaattaactagccctgttgctgcttctgaagagtttgaagatgaagaagaaagtcctgttaatttccccatttactaaagatctacatctcgctttcttgctgtccaatttctattaaaggttcctttgttccctaagtccaactactaaactgggggatattatgaagggccttgagcatctggattctgcctaataaaaaacatttattttcattgcaatgatgtatttaaattatttctgaatattttactaaaaagggaatgtgggaggtcagtgcatttaaaacataaagaaagtaggtaaccacgtgcggaccgagcggccgcaggaacccctagtgatggagttggccactccctctctgcgcgctcgctcgctcactgaggccgggcgaccaaaggtcgcccgacgcccgggctttgcccgggcggcctcagtgagcgagcgagcgcgcagctgcctgca

SEQ ID NO: 42 - DNA, 2108 bp, Artificial sequence
  Sequence of mouse DSD expression vector
ggcagctgcgcgctcgctcgctcactgaggccgcccgggcaaagcccgggcgtcgggcgacctttggtcgcccggcctcagtgagcgagcgagcgcgcagagagggagtggccaactccatcactaggggttcctgcggccgcacgcgtggagctagttattaatagtaatcaattacggggtcattagttcatagcccatatatggagttccgcgttacataacttacggtaaatggcccgcctggctgaccgcccaacgacccccgcccattgacgtcaataatgacgtatgttcccatagtaacgtcaatagggactttccattgacgtcaatgggtggagtatttacggtaaactgcccacttggcagtacatcaagtgtatcatatgccaagtacgccccctattgacgtcaatgacggtaaatggcccgcctggcattatgcccagtacatgaccttatgggactttcctacttggcagtacatctacgtattagtcatcgctattaccatggtgatgcggttttggcagtacatcaatgggcgtggatagcggtttgactcacggggatttccaagtctccaccccattgacgtcaatgggagtttgttttgcaccaaaatcaacgggactttccaaaatgtcgtaacaactccgccccattgacgcaaatgggcggtaggcgtgtacggtgggaggtctatataagcagagctcgtttagtgaaccgtcagatcgcctggagacgccatccacgctgttttgacctccatagaagacaccgggaccgatccagcctccgcggccaccatggatttacttaagcagtctcctgctccagttcccaccaacaaacatttcattcgtctggccgagatggagcagacagtagcagaacaagatgactctctgtcctcacttttgaccaaactaaagaaagtatcaaaagatttggaaaaacaaaaagaaatcactgagttaaaagtcagagagtttgaaaataccaaactacggctccaagaaactcatgccagtgaggtaaagaaagtgaaagcagaggtagaggacttaaggcatgctctagcccaagcacacaaggactcccagagtttaaagtctgaactccaggctcagaaagaagcaaactccagagctccaacaaccacaatgaggaatcttgtagacaggctaaagagccaactagccttgaaagagaagcaacaaaaggcacttagtcgagccctgttggaacttcggtcggaaatgacagcagcagctgaggaacgtataatcgctgtaacttctcaaaaagaggcaaatctcaatgttcaacaagttgttgagcgccatactagagagctaaagtcacaaattgaagatttaaatgaaaatcttttaaaattgaaagaagctcttaaaacaagtaagaacaaagaaaattcactagctgatgatttaaatgaattaaataatgaactgcaaaaaaagcaaaaagcttataataaaatccttagagagaaagatggaattgatcaagaaaatgatgaactgagaagacagattaaaagactgtccagtggactgcagagcaaaactttgatagataacaagcaaagtttaatcgatgaacttcaaaagaaagttaaaaaacttgaaagccaactggaaagaaaggtggatgacgtagacataaagccggtgaaggaaaagtagagatctacatctcgctttcttgctgtccaatttctattaaaggttcctttgttccctaagtccaactactaaactgggggatattatgaagggccttgagcatctggattctgcctaataaaaaacatttattttcattgcaatgatgtatttaaattatttctgaatattttactaaaaagggaatgtgggaggtcagtgcatttaaaacataaagaaagtaggtaaccacgtgcggaccgagcggccgcaggaacccctagtgatggagttggccactccctctctgcgcgctcgctcgctcactgaggccgggcgaccaaaggtcgcccgacgcccgggctttgcccgggcggcctcagtgagcgagcgagcgcgcagctgcctgca

SEQ ID NO: 43 - DNA, 2108 bp, Artificial sequence
  Sequence of human DSD expression vector
ggcagctgcgcgctcgctcgctcactgaggccgcccgggcaaagcccgggcgtcgggcgacctttggtcgcccggcctcagtgagcgagcgagcgcgcagagagggagtggccaactccatcactaggggttcctgcggccgcacgcgtggagctagttattaatagtaatcaattacggggtcattagttcatagcccatatatggagttccgcgttacataacttacggtaaatggcccgcctggctgaccgcccaacgacccccgcccattgacgtcaataatgacgtatgttcccatagtaacgtcaatagggactttccattgacgtcaatgggtggagtatttacggtaaactgcccacttggcagtacatcaagtgtatcatatgccaagtacgccccctattgacgtcaatgacggtaaatggcccgcctggcattatgcccagtacatgaccttatgggactttcctacttggcagtacatctacgtattagtcatcgctattaccatggtgatgcggttttggcagtacatcaatgggcgtggatagcggtttgactcacggggatttccaagtctccaccccattgacgtcaatgggagtttgttttgcaccaaaatcaacgggactttccaaaatgtcgtaacaactccgccccattgacgcaaatgggcggtaggcgtgtacggtgggaggtctatataagcagagctcgtttagtgaaccgtcagatcgcctggagacgccatccacgctgttttgacctccatagaagacaccgggaccgatccagcctccgcggccaccatggatttaatgaaacagtctcccactccagttcctaccaacaagcattttattcgtctggctgagatggaacagacagtagcagaacaagatgactctctttcctcactcttggtcaaactaaagaaagtatcacaagatttggagagacaaagagaaatcactgaattaaaagtaaaagaatttgaaaatatcaaattacagcttcaagaaaaccatgaagatgaagtgaaaaaagtaaaagcggaagtagaggatttaaagtatcttctggaccagtcacaaaaggagtcacagtgtttaaaatctgaacttcaggctcaaaaagaagcaaattcaagagctccaacaactacaatgagaaatctagtagaacggctaaagagccaattagccttgaaggagaaacaacagaaagcacttagtcgggcacttttagaactccgggcagaaatgacagcagctgctgaagaacgtattatttctgcaacttctcaaaaagaggcccatctcaatgttcaacaaatcgttgatcgacatactagagagctaaagacacaagttgaagatttaaatgaaaatcttttaaaattgaaagaagcacttaaaacaagtaaaaacagagaaaactcactaactgataatttgaatgacttaaataatgaactgcaaaagaaacaaaaagcctataataaaatacttagagagaaagaggaaattgatcaagagaatgatgaactgaaaaggcaaattaaaagactaaccagtggattacagggcaaacccctgacagataataaacaaagtctaattgaagaactccaaaggaaagttaaaaaactagagaaccaattagagggaaaggtggaggaagtagacctaaaacctatgaaagaaaagtagagatctacatctcgctttcttgctgtccaatttctattaaaggttcctttgttccctaagtccaactactaaactgggggatattatgaagggccttgagcatctggattctgcctaataaaaaacatttattttcattgcaatgatgtatttaaattatttctgaatattttactaaaaagggaatgtgggaggtcagtgcatttaaaacataaagaaagtaggtaaccacgtgcggaccgagcggccgcaggaacccctagtgatggagttggccactccctctctgcgcgctcgctcgctcactgaggccgggcgaccaaaggtcgcccgacgcccgggctttgcccgggcggcctcagtgagcgagcgagcgcgcagctgcctgca

SEQ ID NO: 44 - DNA, 5132 bp, Artificial sequence
  Sequence of mouse C-terminal expression vector
ggcagctgcgcgctcgctcgctcactgaggccgcccgggcaaagcccgggcgtcgggcgacctttggtcgcccggcctcagtgagcgagcgagcgcgcagagagggagtggccaactccatcactaggggttcctgcggccgcacgcgtggagctagttattaatagtaatcaattacggggtcattagttcatagcccatatatggagttccgcgttacataacttacggtaaatggcccgcctggctgaccgcccaacgacccccgcccattgacgtcaataatgacgtatgttcccatagtaacgtcaatagggactttccattgacgtcaatgggtggagtatttacggtaaactgcccacttggcagtacatcaagtgtatcatatgccaagtacgccccctattgacgtcaatgacggtaaatggcccgcctggcattatgcccagtacatgaccttatgggactttcctacttggcagtacatctacgtattagtcatcgctattaccatggtgatgcggttttggcagtacatcaatgggcgtggatagcggtttgactcacggggatttccaagtctccaccccattgacgtcaatgggagtttgttttgcaccaaaatcaacgggactttccaaaatgtcgtaacaactccgccccattgacgcaaatgggcggtaggcgtgtacggtgggaggtctatataagcagagctcgtttagtgaaccgtcagatcgcctggagacgccatccacgctgttttgacctccatagaagacaccgggaccgatccagcctccgcggccaccatgcaacaacagtccagggaaaaggaagtggaatccctcagaacgcagctgctggacttccaggcacaatctgacgaaaaggctctaattgccaaattgcaccaacatgttgtctctcttcaaattagtgaggccactgccctcggtaagttagagtcagttacgtccaaactccagaagatggaagcctacaatttgcgcttagaacagaaactggatgaaaaagagcaggcgctctactatgctcgtttggaaggtagaaacagagcaaaacacctgcgccaaaccattcagtcgcttcgaagacagttcagtggagctctacccttagcacagcaggaaaagttctccaaaacgatgattcagttgcaaaatgacaaacttaagataatgcaagaaatgaagaattcgcaacaggaacacagaaatatggaaaacaaaacactggagttggaattaaaattaaaaggcttagaagaattgatcagtactttaaaggatgccaggggagcccagaaggtaatcaattggcatgtgaaaatagaagaacttcgcctccaagaacttaagctaaatagagaactagtcaagggtaaagaagaaatcaaatatttgaataatatcatctctgaatatgagcatacaatcaacagtctagaggaagaaattgttcagcaaagcaagttccatgaagaaagacagatggcttgggatcaaagagaagttgagctggaacgccagttagacatttttgatcatcagcaaaatgaaatactcagtgcagcacaaaagtttgaagactctacaggatcaatgccagaccccagcttgcctcttccaaaccaacttgaaattgctctaagaaaaattaaggagaatattcaagtaattcttaaaacacaagcaacttgcaagtcactagaagagaaactaaaagaaaaagaatctgctttacggttggcagagcaaaatattctgtcaagagacaaagtaatcaatgaactgaggcttcgattgcctgccacggctgatcgagaaaaacttatagctgagctagaaagaaaagagctggagccgaaatctcatcacacaatgaaaattgcccaccaaactattgccaacatgcaggcaaggttaaatcacaaggaagaagtattgaagaaataccagcaccttctggagaaggccagagaggagcaaagagaaattgttaagaagcatgaggaagaccttcatgttcttcatcacaaattagaacaacaggccgataattcactcaataaattcagacagacagctcaggatttacttaagcagtctcctgctccagttcccaccaacaaacatttcattcgtctggccgagatggagcagacagtagcagaacaagatgactctctgtcctcacttttgaccaaactaaagaaagtatcaaaagatttggaaaaacaaaaagaaatcactgagttaaaagtcagagagtttgaaaataccaaactacggctccaagaaactcatgccagtgaggtaaagaaagtgaaagcagaggtagaggacttaaggcatgctctagcccaagcacacaaggactcccagagtttaaagtctgaactccaggctcagaaagaagcaaactccagagctccaacaaccacaatgaggaatcttgtagacaggctaaagagccaactagccttgaaagagaagcaacaaaaggcacttagtcgagccctgttggaacttcggtcggaaatgacagcagcagctgaggaacgtataatcgctgtaacttctcaaaaagaggcaaatctcaatgttcaacaagttgttgagcgccatactagagagctaaagtcacaaattgaagatttaaatgaaaatcttttaaaattgaaagaagctcttaaaacaagtaagaacaaagaaaattcactagctgatgatttaaatgaattaaataatgaactgcaaaaaaagcaaaaagcttataataaaatccttagagagaaagatggaattgatcaagaaaatgatgaactgagaagacagattaaaagactgtccagtggactgcagagcaaaactttgatagataacaagcaaagtttaatcgatgaacttcaaaagaaagttaaaaaacttgaaagccaactggaaagaaaggtggatgacgtagacataaagccggtgaaggaaaagagtagtaaagaagaattaattaggtgggaagaaggtaagaaatggcaaaccaaagtagagggactacgaaacagactaaaggagaaggaaggagaagcccacggcctggcaaagcagctgaataccttaaaggaactttttgccaaagctgataaagagaaacttactttgcagaagaaactgaaaacaacaggaatgactgttgaccaggttttaggagtgcgagctttggaatctgaaaaagagttggaagagctaaaaaagaaaaatctggacctagaaaatgacatattatacatgaggacccagcaggctcttccacgagattctgttgtggaagacttacatttacaaaataaataccttcaagaaaaacttcatactttagaaaaaaaactttcaaaggagaaatattctcagtctttgacttcagaaatagagtcagatgatcactgtcaaaaagaacaagaacttcagaaggaaaatttgaagttgtcatctgaaaacatcgagctgaaatttcaacttgaacaagcaaataaagatttgccaagactaaagaatcaagtgaaagatttgaaggaaatgtgtgaatttcttaagaaaggaaaactggaacttgagcggaagcttggtcaggtcagaggggctggtagaagtgggaagacaatcccagaactagaaaaaaccattgggttaatgaagaaagtagttgaaaaagtccaaagagaaaatgaacaattgaaaaaggcatcaggaatactgactagtgaaaaaatggctactattgaggaagaaaatagaaacttaaaggctgaactagaaaagcttaaagctcactttggacgtcagttgagtatgcagtttgaatctaagaacaaaggtactgagaaaattgttgccgaaaatgaacggcttcggaaagaacttaagaaagaaatagaagcctctgagaaactgcggatagctaagaacaacttagagctggtgaacgacaagatggcagctcaactcgaagaaactgggaagagactacagtttgcagaaagtagagccccacagctggaaggtgctgacagcaagagctggaagtcaattgtggtctcaagagtgtatgagaccaagatgaaagagcttgaaagtgacattgccaaaaagaatcaaagtatcactgaccttaaacagcttgtaagagaagcaacagagagagaacagaaagctaagaaatacactgaagaccttgaacaacagattgagatcctcaaaaatgttcctgaaggtgccgagacagagcaagagcttatacgggaactccagcttcttagattagccaataatcagatggataaagaaagggcagaattaatccatcagatagaaattaacaaggaccaaaccagagctgacagtagcatacctgattctgatcaactaaaggaaaagataaatgacctggagacacaactcagaaagttggagctagaaaagcaacattcgaaggaggaagttaaaaagctgaaaaaagaactggaaaattttgatccttcattttttgaagaaattgaagacctgaagtataattataaggaagaagtgaaaaagaatatcctattagaagagaagctaaaaaaactgtcggaacagtttggatttgaactgcctagtcctcttgctgcttctgaacactcggaagatggagaaagtcctcatagtttccctatttattagagatctacatctcgctttcttgctgtccaatttctattaaaggttcctttgttccctaagtccaactactaaactgggggatattatgaagggccttgagcatctggattctgcctaataaaaaacatttattttcattgcaatgatgtatttaaattatttctgaatattttactaaaaagggaatgtgggaggtcagtgcatttaaaacataaagaaagtaggtaaccacgtgcggaccgagcggccgcaggaacccctagtgatggagttggccactccctctctgcgcgctcgctcgctcactgaggccgggcgaccaaaggtcgcccgacgcccgggctttgcccgggcggcctcagtgagcgagcgagcgcgcagctgcctgca

SEQ ID NO: 45 - DNA, 5132 bp, Artificial sequence
  Sequence of human C-terminal expression vector
ggcagctgcgcgctcgctcgctcactgaggccgcccgggcaaagcccgggcgtcgggcgacctttggtcgcccggcctcagtgagcgagcgagcgcgcagagagggagtggccaactccatcactaggggttcctgcggccgcacgcgtggagctagttattaatagtaatcaattacggggtcattagttcatagcccatatatggagttccgcgttacataacttacggtaaatggcccgcctggctgaccgcccaacgacccccgcccattgacgtcaataatgacgtatgttcccatagtaacgtcaatagggactttccattgacgtcaatgggtggagtatttacggtaaactgcccacttggcagtacatcaagtgtatcatatgccaagtacgccccctattgacgtcaatgacggtaaatggcccgcctggcattatgcccagtacatgaccttatgggactttcctacttggcagtacatctacgtattagtcatcgctattaccatggtgatgcggttttggcagtacatcaatgggcgtggatagcggtttgactcacggggatttccaagtctccaccccattgacgtcaatgggagtttgttttgcaccaaaatcaacgggactttccaaaatgtcgtaacaactccgccccattgacgcaaatgggcggtaggcgtgtacggtgggaggtctatataagcagagctcgtttagtgaaccgtcagatcgcctggagacgccatccacgctgttttgacctccatagaagacaccgggaccgatccagcctccgcggccaccatgcaacaatctagggacaaggaagtagagtccctcagaatgcaactgctagactatcaggcacagtctgatgaaaagtcgctcattgccaagttgcaccaacataatgtctctcttcaactgagtgaggctactgctcttggtaagttggagtcaattacatctaaactgcagaagatggaggcctacaacttgcgcttagagcagaaacttgatgaaaaagaacaggctctctattatgctcgtttggagggaagaaacagagcaaaacatctgcgccaaacaattcagtctctacgacgacagtttagtggagctttacccttggcacaacaggaaaagttctccaaaacaatgattcaactacaaaatgacaaacttaagataatgcaagaaatgaaaaattctcaacaagaacatagaaatatggagaacaaaacattggagatggaattaaaattaaagggcctggaagagttaataagcactttaaaggataccaaaggagcccaaaaggtaatcaactggcatatgaaaatagaagaacttcgtcttcaagaacttaaactaaatcgggaattagtcaaggataaagaagaaataaaatatttgaataacataatttctgaatatgaacgtacaatcagcagtcttgaagaagaaattgtgcaacagaacaagtttcatgaagaaagacaaatggcctgggatcaaagagaagttgacctggaacgccaactagacatttttgaccgtcagcaaaatgaaatactaaatgcggcacaaaagtttgaagaagctacaggatcaatccctgaccctagtttgccccttccaaatcaacttgagatcgctctaaggaaaattaaggagaacattcgaataattctagaaacacgggcaacttgcaaatcactagaagagaaactaaaagagaaagaatctgctttaaggttagcagaacaaaatatactgtcaagagacaaagtaatcaatgaactgaggcttcgattgcctgccactgcagaaagagaaaagctcatagctgagctaggcagaaaagagatggaaccaaaatctcaccacacattgaaaattgctcatcaaaccattgcaaacatgcaagcaaggttaaatcaaaaagaagaagtattaaagaagtatcaacgtcttctagaaaaagccagagaggagcaaagagaaattgtgaagaaacatgaggaagaccttcatattcttcatcacagattagaactacaggctgatagttcactaaataaattcaaacaaacggcttgggatttaatgaaacagtctcccactccagttcctaccaacaagcattttattcgtctggctgagatggaacagacagtagcagaacaagatgactctctttcctcactcttggtcaaactaaagaaagtatcacaagatttggagagacaaagagaaatcactgaattaaaagtaaaagaatttgaaaatatcaaattacagcttcaagaaaaccatgaagatgaagtgaaaaaagtaaaagcggaagtagaggatttaaagtatcttctggaccagtcacaaaaggagtcacagtgtttaaaatctgaacttcaggctcaaaaagaagcaaattcaagagctccaacaactacaatgagaaatctagtagaacggctaaagagccaattagccttgaaggagaaacaacagaaagcacttagtcgggcacttttagaactccgggcagaaatgacagcagctgctgaagaacgtattatttctgcaacttctcaaaaagaggcccatctcaatgttcaacaaatcgttgatcgacatactagagagctaaagacacaagttgaagatttaaatgaaaatcttttaaaattgaaagaagcacttaaaacaagtaaaaacagagaaaactcactaactgataatttgaatgacttaaataatgaactgcaaaagaaacaaaaagcctataataaaatacttagagagaaagaggaaattgatcaagagaatgatgaactgaaaaggcaaattaaaagactaaccagtggattacagggcaaacccctgacagataataaacaaagtctaattgaagaactccaaaggaaagttaaaaaactagagaaccaattagagggaaaggtggaggaagtagacctaaaacctatgaaagaaaagaatgctaaagaagaattaattaggtgggaagaaggtaaaaagtggcaagccaaaatagaaggaattcgaaacaagttaaaagagaaagagggggaagtctttactttaacaaagcagttgaatactttgaaggatctttttgccaaagccgataaagagaaacttactttgcagaggaaactaaaaacaactggcatgactgttgatcaggttttgggaatacgagctttggagtcagaaaaagaattggaagaattaaaaaagagaaatcttgacttagaaaatgatatattgtatatgagggcccaccaagctcttcctcgagattctgttgtagaagatttacatttacaaaatagatacctccaagaaaaacttcatgctttagaaaaacagttttcaaaggatacatattctaagccttcaatttcaggaatagagtcagatgatcattgtcagagagaacaggagcttcagaaggaaaacttgaagttgtcatctgaaaatattgaactgaaatttcagcttgaacaagcaaataaagatttgccaagattaaagaatcaagtcagagatttgaaggaaatgtgtgaatttcttaagaaagaaaaagcagaagttcagcggaaacttggccatgttagagggtctggtagaagtggaaagacaatcccagaactggaaaaaaccattggtttaatgaaaaaagtagttgaaaaagtccagagagaaaatgaacagttgaaaaaagcatcaggaatattgactagtgaaaaaatggctaatattgagcaggaaaatgaaaaattgaaggctgaattagaaaaacttaaagctcatcttgggcatcagttgagcatgcactatgaatccaagaccaaaggcacagaaaaaattattgctgaaaatgaaaggcttcgtaaagaacttaaaaaagaaactgatgctgcagagaaattacggatagcaaagaataatttagagatattaaatgagaagatgacagttcaactagaagagactggtaagagattgcagtttgcagaaagcagaggtccacagcttgaaggtgctgacagtaagagctggaaatccattgtggttacaagaatgtatgaaaccaagttaaaagaattggaaactgatattgccaaaaaaaatcaaagcattactgaccttaaacagcttgtaaaagaagcaacagagagagaacaaaaagttaacaaatacaatgaagaccttgaacaacagattaagattcttaaacatgttcctgaaggtgctgagacagagcaaggccttaaacgggagcttcaagttcttagattagctaatcatcagctggataaagagaaagcagaattaatccatcagatagaagctaacaaggaccaaagtggagctgaaagcaccatacctgatgctgatcaactaaaggaaaaaataaaagatctagagacacagctcaaaatgtcagatctagaaaagcagcatttgaaggaggaaataaagaagctgaaaaaagaactggaaaattttgatccttcattttttgaagaaattgaagatcttaagtataattacaaggaagaagtgaagaagaatattctcttagaagagaaggtaaaaaaactttcagaacaattgggagttgaattaactagccctgttgctgcttctgaagagtttgaagatgaagaagaaagtcctgttaatttccccatttactaaagatctacatctcgctttcttgctgtccaatttctattaaaggttcctttgttccctaagtccaactactaaactgggggatattatgaagggccttgagcatctggattctgcctaataaaaaacatttattttcattgcaatgatgtatttaaattatttctgaatattttactaaaaagggaatgtgggaggtcagtgcatttaaaacataaagaaagtaggtaaccacgtgcggaccgagcggccgcaggaacccctagtgatggagttggccactccctctctgcgcgctcgctcgctcactgaggccgggcgaccaaaggtcgcccgacgcccgggctttgcccgggcggcctcagtgagcgagcgagcgcgcagctgcctgca